European Patent Application EP 4 137 570 A1, published February 22, 2023. Title: OPTIMIZED FACTOR VIII GENES. Applicant: BIOVERATIV THERAPEUTICS INC. Application To be assigned. The sequence listing filed with the application follows.

SEQUENCE LISTING (103 sequences)

SEQ ID NO: 1 - DNA, 4374 bp, Artificial Sequence
  coFVIII-5
atgcaaatcgaactgagcacctgtttcttcctctgcctgctgagattctgtttctccgcgacccgccgatactacctgggagcagtggagctctcctgggattacatgcagagcgaccttggggagctgcccgtggatgccaggttccctccccgggtgccaaagtcgtttccgttcaacacctccgtggtgtacaagaaaactctgttcgtggagttcaccgaccacctgttcaatatcgccaagcccagacctccctggatggggctgttgggacctaccatccaagcggaggtgtacgacactgtggtcatcactctgaagaacatggcctcgcatcccgtgtccctgcacgccgtgggagtgtcttactggaaagcgtccgagggggccgaatacgacgaccagacctcgcagagagaaaaggaagatgacaaggtgttcccaggaggatcgcacacctacgtgtggcaagtgttgaaggagaacggcccaatggcctccgacccgctgtgcctgacctactcgtacctgtcccacgtggacctcgtgaaggacctcaactcgggactgattggagccctgctggtctgcagggaaggctcactggcgaaagaaaagactcagaccttgcacaagttcattctgctgttcgctgtgttcgacgaggggaagtcgtggcacagcgagactaagaactccctgatgcaagatagagatgccgcctccgcccgggcctggcctaagatgcacaccgtgaacggttacgtgaaccgctccctccctggcctgattggatgccaccggaagtccgtgtactggcacgtgatcgggatggggaccacccccgaggtgcacagcatcttcctggaaggtcacacatttctcgtgcgcaaccaccggcaggcctccctggaaatcagccccattaccttcctcactgcccagactctgctgatggacctgggacagttcctgctgttctgccatatctcctcccaccaacatgacggaatggaggcatacgtgaaggtcgattcctgccctgaggaaccccagctccgcatgaagaacaatgaggaagccgaggactacgacgacgacctgacggatagcgagatggatgtggtccggttcgatgacgataacagcccttccttcatccaaattcgctcggtggcaaagaagcaccccaagacctgggtgcattacattgcggcggaagaagaggactgggattatgccccgcttgtcctcgctcctgacgaccggagctacaagagccagtacctgaacaacggtccacagaggatcggtagaaagtacaagaaggtccgcttcatggcctataccgacgaaaccttcaaaactagagaggccatccaacacgaatccggcatcctgggcccgctcttgtacggagaagtcggcgacacccttctcattatcttcaagaaccaggcttcccggccgtacaacatctatccgcatgggatcactgacgtgcgcccactgtactcgcggcgcctgcccaagggtgtcaaacacctgaaggattttccgatccttccgggagaaatcttcaagtacaagtggaccgtgaccgtggaagatggcccaactaagtctgaccctagatgcctcacccgctactactcatccttcgtcaacatggagcgcgacctggccagcggactgatcggcccgctgctgatttgctacaaggaatcagtggaccaacggggaaaccagatcatgtcggataagaggaacgtcatcctcttctccgtgtttgacgaaaaccggtcgtggtacctgactgaaaacatccagcggttcctccccaaccccgcgggcgtgcagctggaagatcctgagtttcaggcatcaaacatcatgcactccattaacggctacgtgttcgattcgctgcagctgagcgtgtgtctgcacgaagtggcctactggtacatcctgtccattggtgcccagactgacttcctgtccgtgtttttctccggctacacgttcaagcacaagatggtgtacgaggacaccctgaccctcttccctttttccggcgaaactgtgtttatgagcatggagaatcccggcctgtggatcttgggctgccacaacagcgacttccgtaacagaggaatgactgcgctgctcaaggtgtccagctgcgacaagaacaccggagactattatgaggactcatacgaggacatctccgcctacctcctgtccaagaataacgccattgaacctcggagcttcagccagaacccacccgtgcttaagagacatcaacgggagatcactaggaccaccctgcagtcagaccaggaggaaatcgactacgatgacaccatctcggtcgagatgaagaaggaggactttgacatctacgacgaagatgaaaaccagagcccgaggtcgttccaaaagaaaacccgccactactttattgctgctgtcgagcggctgtgggactacggaatgtcgtcctcgccgcacgtgctccgcaaccgagcccagagcggctcggtgccgcaattcaagaaggtcgtgttccaggagttcactgacgggagcttcactcagcctttgtaccggggagaactcaatgaacatctcggcctcctcggaccttacatcagagcagaagtggaagataacatcatggtcactttccgtaaccaagccagccgcccgtactcgttctactcctccctcatttcttacgaagaggaccagcggcagggcgcagaaccgcgcaagaacttcgtgaagcccaacgaaaccaagacctacttctggaaagtgcagcatcatatggccccgactaaggacgagtttgactgcaaagcctgggcctacttctccgatgtggacttggagaaggacgtccactccggcctcatcggtcccctgctcgtgtgccataccaataccctgaaccccgcacacggtcgccaggtcaccgtgcaggagttcgctctgttcttcactatcttcgacgaaactaagtcctggtacttcaccgagaacatggagaggaactgcagagccccctgtaacatccagatggaggacccgacgttcaaggaaaactaccggttccacgccattaacggatacatcatggatacgctgccgggtcttgtgatggcccaggatcaacggatcagatggtacttattgtcgatgggcagcaacgagaacatccactctattcacttctccggtcatgtgttcactgtgcggaagaaggaagagtacaagatggccctgtacaacctttatcccggagtgttcgaaactgtggaaatgctgccgtcgaaggccggcatttggcgcgtggagtgtttgattggagaacatctccatgcggggatgtcaaccctgttcctggtgtatagcaacaagtgccagactccgcttgggatggcgtcaggacacattagggatttccagatcactgcgtccggccagtacggccaatgggcccctaagctggcccgcctgcattactccggatccattaacgcctggtcaaccaaggagccattctcctggatcaaggtggaccttctggcccccatgattatccacggaattaagacccagggggcccggcagaagttctcctcactgtacatcagccagttcataatcatgtactccctggacggaaagaagtggcaaacctacagggggaacagcaccggcacactgatggtctttttcggaaatgtggactcctccgggattaagcataacatcttcaaccctccgattatcgctcggtacattagacttcaccctacccactacagcattcgctccaccctgcggatggaactgatgggctgcgatctgaactcgtgcagcatgccgttgggaatggagtccaaagcaatttccgacgcgcagatcaccgcctcgtcctactttaccaacatgttcgccacgtggtcaccgtccaaggcccggctgcacctccagggaagatccaacgcatggcggccacaggtcaacaaccctaaggagtggctccaggtggacttccagaaaaccatgaaggtcaccggagtcacaacccagggagtgaagtcgctgctgacttctatgtacgtcaaggagttcctgatctccagcagccaggacgggcaccagtggaccctgttcttccaaaatggaaaggtcaaggtgtttcagggcaatcaggattcattcaccccggtggtgaactcccttgatccacccctcctgacccgctaccttcgcatccacccacagtcctgggtgcaccagatcgcgctgaggatggaggtcctgggatgcgaagcccaggacctgtactga

SEQ ID NO: 2 - DNA, 4374 bp, Artificial Sequence
  coFVIII-4
atgcagatcgagctgagcacgtgcttcttcctgtgcctgctgaggttctgcttcagcgccaccaggaggtactacctgggcgccgtggagctgagctgggactacatgcagagcgacctgggcgagctgcccgtggacgccaggttcccccccagggtgcccaagagcttccccttcaacacgagcgtggtgtacaagaagaccctgttcgtggagttcaccgaccatctgttcaatatcgccaagcccaggcccccctggatggggctgctggggcccacgatccaggccgaggtgtacgacaccgtggtcatcaccctgaagaacatggccagccaccccgtgagcctgcacgccgtgggcgtgagctactggaaggccagcgagggcgccgagtacgacgaccagaccagccagagggagaaggaggacgacaaggtgttccccggcggcagccacacctacgtgtggcaggtgctgaaggagaatgggcccatggccagcgaccccctgtgcctgacctactcttacctgagccacgtggatctggtgaaggacctgaacagcggcctgatcggcgccctgctggtgtgcagggagggcagcctggccaaggagaagacccagaccctgcacaagttcatcctgctgttcgccgtgttcgacgagggcaagagctggcacagcgagaccaagaacagcctgatgcaggatagggacgccgccagcgccagggcctggcccaagatgcacaccgtgaacggctacgtgaacaggtctctgcccggcctgatcggctgccacaggaagagcgtgtactggcacgtgatcggcatggggaccacccccgaggtgcacagcatcttcctggagggccacacgttcctggtgaggaatcacaggcaggccagcctggagatcagcccgatcaccttcctgaccgcccagaccctgctgatggacctggggcagttcctgctgttctgccatatcagctctcaccagcacgacggcatggaggcctacgtgaaggtggatagctgccccgaggagccccagctgaggatgaagaacaacgaggaggccgaggactacgacgacgacctgaccgacagcgagatggacgtggtgaggttcgacgacgacaatagcccgagcttcatccagatcaggagcgtggccaagaagcaccccaagacctgggtgcattacatcgccgccgaggaggaggattgggactacgcccccctggtgctggcccccgacgacaggtcttacaagagccagtacctgaacaacgggccccagaggatcggcaggaagtacaagaaggtgaggttcatggcctacaccgacgagaccttcaagaccagggaggcgatccagcacgagagcgggatcctggggcccctgctgtacggcgaggtgggcgacacgctgctgatcatcttcaagaaccaggccagcaggccgtacaatatctacccccacgggatcaccgacgtgaggcccctgtactctaggaggctgcccaagggcgtgaagcacctgaaggacttccccatcctgcccggcgagatcttcaagtacaagtggaccgtgaccgtggaggacgggcccacgaagagcgaccccaggtgcctgaccaggtactacagctctttcgtgaacatggagagggacctggccagcggcctgatcgggcccctgctgatctgctacaaggagagcgtggatcagaggggcaaccagatcatgagcgacaagaggaacgtgatcctgttcagcgtgttcgacgagaataggtcttggtacctgaccgagaatatccagaggttcctgcccaaccccgccggcgtgcagctggaggatcccgagttccaggccagcaacatcatgcacagcatcaacggctacgtgttcgacagcctgcagctgagcgtgtgcctgcacgaggtggcctactggtacatcctgagcatcggcgcccagaccgacttcctgagcgtgttcttcagcggctacaccttcaagcacaagatggtgtacgaggataccctgaccctgttccccttcagcggcgagaccgtgttcatgagcatggagaaccccggcctgtggatcctgggctgccataactccgacttcaggaataggggcatgaccgccctgctgaaggtgagctcttgcgacaagaacaccggcgactactacgaggatagctacgaggatatcagcgcctacctgctgagcaagaacaacgccatcgagcccaggtctttcagccagaacccccccgtgctgaagaggcaccagagggagatcaccaggacgaccctgcagagcgaccaggaggagatcgactacgacgacacgatcagcgtggagatgaagaaggaggatttcgacatctacgacgaggacgagaatcagagccccaggtctttccagaagaagaccaggcattacttcatcgccgccgtggagaggctgtgggactacggcatgagcagctctccccacgtgctgaggaatagggcccagagcggcagcgtgccccagttcaagaaggtggtgttccaggagttcaccgacggcagcttcacccagcccctgtacaggggcgagctgaacgagcacctgggcctgctggggccctacatcagggccgaggtggaggataacatcatggtgaccttcaggaatcaggccagcaggccctatagcttctatagctctctgatcagctacgaggaggatcagaggcagggcgccgagcccaggaagaacttcgtgaagcccaacgagaccaagacctacttctggaaggtgcagcaccacatggcccccacgaaggacgagttcgactgcaaggcctgggcctacttcagcgacgtggatctggagaaggacgtgcacagcggcctgatcgggcccctgctggtgtgccacaccaacaccctgaaccccgcccacggcaggcaggtgaccgtgcaggagttcgccctgttcttcaccatcttcgacgagaccaagagctggtacttcaccgagaatatggagaggaattgcagggccccctgcaatatccagatggaggacccgaccttcaaggagaattacaggttccacgccatcaacggctacatcatggacacgctgcccggcctggtcatggcccaggatcagaggatcaggtggtatctgctgagcatggggagcaacgagaatatccacagcatccacttcagcggccacgtgttcaccgtgaggaagaaggaggagtacaagatggccctgtacaatctgtaccccggcgtgttcgagaccgtggagatgctgcccagcaaggccgggatctggagggtggagtgcctgatcggcgagcacctgcacgccggcatgagcacgctgttcctggtgtactctaacaagtgccagacccccctggggatggccagcggccacatcagggacttccagatcaccgccagcggccagtacggccagtgggcccccaagctggccaggctgcactattccggaagcatcaacgcctggagcacgaaggagcccttcagctggatcaaggtggatctgctggcccccatgatcatccacgggatcaagacccagggcgccaggcagaagttcagctctctgtatatcagccagttcatcatcatgtactctctggacggcaagaagtggcagacctacaggggcaacagcaccggcacgctgatggtgttcttcggcaacgtggactctagcgggatcaagcacaatatcttcaacccccccatcatcgccaggtacatcaggctgcaccccacccattactctatcaggtctaccctgaggatggagctgatgggctgcgacctgaacagctgcagcatgcccctggggatggagagcaaggccatcagcgacgcccagatcaccgccagctcttacttcaccaacatgttcgccacctggagcccgagcaaggccaggctgcacctgcagggcaggtctaacgcctggaggccccaggtgaacaaccccaaggagtggctgcaggtggatttccagaagaccatgaaggtgaccggcgtgaccacgcagggcgtgaagagcctgctgaccagcatgtacgtgaaggagttcctgatcagctctagccaggacggccaccagtggaccctgttcttccagaacggcaaggtgaaggtgttccagggcaaccaggatagcttcacccccgtggtgaacagcctggacccccccctgctgaccaggtatctgaggatccacccccagagctgggtgcaccagatcgccctgaggatggaggtgctgggctgcgaggcccaggatctgtattga

SEQ ID NO: 3 - DNA, 4374 bp, Artificial Sequence
  coFVIII-52
atgcaaatcgaactgagcacctgtttcttcctctgcctgctgagattctgtttctccgcgacccgccgatactacctgggagcagtggagctctcctgggattacatgcagagcgaccttggggagctgcccgtggatgccaggttccctccccgggtgccaaagtcgtttccgttcaacacctccgtggtgtacaagaaaactctgttcgtggagttcaccgaccacctgttcaatatcgccaagcccagacctccctggatggggctgttgggacctaccatccaagcggaggtgtacgacactgtggtcatcactctgaagaacatggcctcgcatcccgtgtccctgcacgccgtgggagtgtcttactggaaagcgtccgagggggccgaatacgacgaccagacctcgcagagagaaaaggaagatgacaaggtgttcccaggaggatcgcacacctacgtgtggcaagtgttgaaggagaacggcccaatggcctccgacccgctgtgcctgacctactcgtacctgtcccacgtggacctcgtgaaggacctcaactcgggactgattggagccctgctggtctgcagggaaggctcactggcgaaagaaaagactcagaccttgcacaagttcattctgctgttcgctgtgttcgacgaggggaagtcgtggcacagcgagactaagaactccctgatgcaagatagagatgccgcctccgcccgggcctggcctaagatgcacaccgtgaacggttacgtgaaccgctccctccctggcctgattggatgccaccggaagtccgtgtactggcacgtgatcgggatggggaccacccccgaggtgcacagcatcttcctggaaggtcacacatttctcgtgcgcaaccaccggcaggcctccctggaaatcagccccattaccttcctcactgcccagactctgctgatggacctgggacagttcctgctgttctgccatatctcctcccaccaacatgacggaatggaggcatacgtgaaggtcgattcctgccctgaggaaccccagctccgcatgaagaacaatgaggaagccgaggactacgacgacgacctgacggatagcgagatggatgtggtccggttcgatgacgataacagcccttccttcatccaaattcgctcggtggcaaagaagcaccccaagacctgggtgcattacattgcggcggaagaagaggactgggattatgccccgcttgtcctcgctcctgacgaccggagctacaagagccagtacctgaacaacggtccacagaggatcggtagaaagtacaagaaggtccgcttcatggcctataccgacgaaaccttcaaaactagagaggccatccaacacgaatccggcatcctgggcccgctcttgtacggagaagtcggcgacacccttctcattatcttcaagaaccaggcttcccggccgtacaacatctatccgcatgggatcactgacgtgcgcccactgtactcgcggcgcctgcccaagggtgtcaaacacctgaaggattttccgatccttccgggagaaatcttcaagtacaagtggaccgtgaccgtggaagatggcccaactaagtctgaccctagatgcctcacccgctactactcatccttcgtcaacatggagcgcgacctggccagcggactgatcggcccgctgctgatttgctacaaggaatcagtggaccaacggggaaaccagatcatgtcggataagaggaacgtcatcctcttctccgtgtttgacgaaaaccggtcgtggtacctgaccgagaacatccagaggttcctgcccaaccctgctggggtgcagctggaggaccccgagttccaggccagcaacatcatgcacagcatcaatggctacgtgttcgacagcctgcagctgagcgtgtgcctgcacgaggtggcctactggtacatcctgagcatcggcgcccagaccgacttcctgagcgtgttcttctctggctacaccttcaagcacaagatggtgtatgaggacaccctgaccctgttccccttcagcggggagactgtcttcatgagcatggagaaccctggcctgtggatcctgggctgccacaacagcgacttcaggaacaggggcatgactgccctgctgaaagtctccagctgtgacaagaacaccggggactactacgaggacagctacgaggacatcagcgcctacctgctgagcaagaacaatgccatcgagcccaggagcttctctcagaaccccccagtgctgaagaggcaccagagggagatcaccaggaccaccctgcagtctgaccaggaggagatcgactatgatgacaccatcagcgtggagatgaagaaggaggacttcgacatctacgacgaggacgagaaccagagccccaggagcttccagaagaagaccaggcactacttcattgctgctgtggagaggctgtgggactatggcatgtccagcagcccccatgtgctgaggaacagggcccagtctggcagcgtgccccagttcaagaaagtcgtgttccaggagttcaccgacggcagcttcacccagcccctgtacagaggggagctgaacgagcacctgggcctgctgggcccctacatcagggccgaggtggaggacaacatcatggtgaccttcaggaaccaggccagcaggccctacagcttctacagcagcctgatcagctacgaggaggaccagaggcagggggctgagcccaggaagaactttgtgaagcccaatgaaaccaagacctacttctggaaggtgcagcaccacatggcccccaccaaggacgagttcgactgcaaggcctgggcctacttctctgacgtggacctggagaaggacgtgcactctggcctgattggccccctgctggtgtgccacaccaacaccctgaaccctgcccatggcaggcaggtgactgtgcaggagttcgccctgttcttcaccatcttcgatgaaaccaagagctggtacttcactgagaacatggagaggaactgcagggccccctgcaacatccagatggaggaccccaccttcaaggagaactacaggttccatgccatcaatggctacatcatggacaccctgcctggcctggtcatggcccaggaccagaggatcaggtggtatctgctgagcatgggcagcaacgagaacatccacagcatccacttctctggccacgtgttcactgtgaggaagaaggaggagtacaagatggccctgtacaacctgtaccctggggtgttcgaaaccgtggagatgctgcccagcaaggccggcatctggagggtggagtgcctgattggggagcacctgcacgccggcatgagcaccctgttcctggtgtacagcaacaagtgccagacccccctgggcatggcctctggccacatcagggacttccagatcactgcctctggccagtacggccagtgggcccccaagctggccaggctgcactactccggaagcatcaatgcctggagcaccaaggagcccttcagctggatcaaagtggacctgctggcccccatgatcatccacggcatcaagacccagggggccaggcagaagttctccagcctgtacatcagccagttcatcatcatgtacagcctggacggcaagaagtggcagacctacaggggcaacagcaccggcaccctgatggtgttcttcggcaacgtggacagcagcggcatcaagcacaacatcttcaacccccccatcatcgccagatacatcaggctgcaccccacccactacagcatcaggagcaccctgaggatggagctgatgggctgtgacctgaacagctgcagcatgcccctgggcatggagagcaaggccatctctgacgcccagatcactgcctccagctacttcaccaacatgtttgccacctggagccccagcaaggccaggctgcacctgcagggcaggagcaatgcctggaggccccaggtcaacaaccccaaggagtggctgcaggtggacttccagaagaccatgaaggtgactggggtgaccacccagggggtgaagagcctgctgaccagcatgtacgtgaaggagttcctgatctccagcagccaggacggccaccagtggaccctgttcttccagaatggcaaggtgaaggtgttccagggcaaccaggacagcttcacccctgtggtcaacagcctggacccccccctgctgaccagatacctgaggatccacccccagagctgggtgcaccagatcgccctgaggatggaggtgctgggctgtgaggcccaggacctgtactga

SEQ ID NO: 4 - DNA, 4374 bp, Artificial Sequence
  coFVIII-62
atgcagattgagctgtccacttgtttcttcctgtgcctcctgcgcttctgtttctccgccactcgccggtactaccttggagccgtggagctttcatgggactacatgcagagcgacctgggcgaactccccgtggatgccagattccccccccgcgtgccaaagtccttcccctttaacacctccgtggtgtacaagaaaaccctctttgtcgagttcactgaccacctgttcaacatcgccaagccgcgcccaccttggatgggcctcctgggaccgaccattcaagctgaagtgtacgacaccgtggtgatcaccctgaagaacatggcgtcccaccccgtgtccctgcatgcggtcggagtgtcctactggaaggcctccgaaggagctgagtacgacgaccagactagccagcgggaaaaggaggacgataaagtgttcccgggcggctcgcatacttacgtgtggcaagtcctgaaggaaaacggacctatggcatccgatcctctgtgcctgacttactcctacctttcccatgtggacctcgtgaaggacctgaacagcgggctgattggtgcacttctcgtgtgccgcgaaggttcgctcgctaaggaaaagacccagaccctccataagttcatccttttgttcgctgtgttcgatgaaggaaagtcatggcattccgaaactaagaactcgctgatgcaggaccgggatgccgcctcagcccgcgcctggcctaaaatgcatacagtcaacggatacgtgaatcggtcactgcccgggctcatcggttgtcacagaaagtccgtgtactggcacgtcatcggcatgggcactacgcctgaagtgcactccatcttcctggaagggcacaccttcctcgtgcgcaaccaccgccaggcctctctggaaatctccccgattacctttctgaccgcccagactctgctcatggacctggggcagttccttctcttctgccacatctccagccatcagcacgacggaatggaggcctacgtgaaggtggactcatgcccggaagaacctcagttgcggatgaagaacaacgaggaggccgaggactatgacgacgatttgactgactccgagatggacgtcgtgcggttcgatgacgacaacagccccagcttcatccagattcgcagcgtggccaagaagcaccccaaaacctgggtgcactacatcgcggccgaggaagaagattgggactacgccccgttggtgctggcacccgatgaccggtcgtacaagtcccagtatctgaacaatggtccgcagcggattggcagaaagtacaagaaagtgcggttcatggcgtacactgacgaaacgtttaagacccgggaggccattcaacatgagagcggcattctgggaccactgctgtacggagaggtcggcgataccctgctcatcatcttcaaaaaccaggcctcccggccttacaacatctaccctcacggaatcaccgacgtgcggccactctactcgcggcgcctgccgaagggcgtcaagcacctgaaagacttccctatcctgccgggcgaaatcttcaagtataagtggaccgtcaccgtggaggacgggcccaccaagagcgatcctaggtgtctgactcggtactactccagcttcgtgaacatggaacgggacctggcatcgggactcattggaccgctgctgatctgctacaaagagtcggtggatcaacgcggcaaccagatcatgtccgacaagcgcaacgtgatcctgttctccgtgtttgatgaaaacagatcctggtacctgaccgagaacatccagaggttcctgcccaaccctgctggggtgcagctggaggaccccgagttccaggccagcaacatcatgcacagcatcaatggctacgtgttcgacagcctgcagctgagcgtgtgcctgcacgaggtggcctactggtacatcctgagcatcggcgcccagaccgacttcctgagcgtgttcttctctggctacaccttcaagcacaagatggtgtatgaggacaccctgaccctgttccccttcagcggggagactgtcttcatgagcatggagaaccctggcctgtggatcctgggctgccacaacagcgacttcaggaacaggggcatgactgccctgctgaaagtctccagctgtgacaagaacaccggggactactacgaggacagctacgaggacatcagcgcctacctgctgagcaagaacaatgccatcgagcccaggagcttctctcagaaccccccagtgctgaagaggcaccagagggagatcaccaggaccaccctgcagtctgaccaggaggagatcgactatgatgacaccatcagcgtggagatgaagaaggaggacttcgacatctacgacgaggacgagaaccagagccccaggagcttccagaagaagaccaggcactacttcattgctgctgtggagaggctgtgggactatggcatgtccagcagcccccatgtgctgaggaacagggcccagtctggcagcgtgccccagttcaagaaagtcgtgttccaggagttcaccgacggcagcttcacccagcccctgtacagaggggagctgaacgagcacctgggcctgctgggcccctacatcagggccgaggtggaggacaacatcatggtgaccttcaggaaccaggccagcaggccctacagcttctacagcagcctgatcagctacgaggaggaccagaggcagggggctgagcccaggaagaactttgtgaagcccaatgaaaccaagacctacttctggaaggtgcagcaccacatggcccccaccaaggacgagttcgactgcaaggcctgggcctacttctctgacgtggacctggagaaggacgtgcactctggcctgattggccccctgctggtgtgccacaccaacaccctgaaccctgcccatggcaggcaggtgactgtgcaggagttcgccctgttcttcaccatcttcgatgaaaccaagagctggtacttcactgagaacatggagaggaactgcagggccccctgcaacatccagatggaggaccccaccttcaaggagaactacaggttccatgccatcaatggctacatcatggacaccctgcctggcctggtcatggcccaggaccagaggatcaggtggtatctgctgagcatgggcagcaacgagaacatccacagcatccacttctctggccacgtgttcactgtgaggaagaaggaggagtacaagatggccctgtacaacctgtaccctggggtgttcgaaaccgtggagatgctgcccagcaaggccggcatctggagggtggagtgcctgattggggagcacctgcacgccggcatgagcaccctgttcctggtgtacagcaacaagtgccagacccccctgggcatggcctctggccacatcagggacttccagatcactgcctctggccagtacggccagtgggcccccaagctggccaggctgcactactccggaagcatcaatgcctggagcaccaaggagcccttcagctggatcaaagtggacctgctggcccccatgatcatccacggcatcaagacccagggggccaggcagaagttctccagcctgtacatcagccagttcatcatcatgtacagcctggacggcaagaagtggcagacctacaggggcaacagcaccggcaccctgatggtgttcttcggcaacgtggacagcagcggcatcaagcacaacatcttcaacccccccatcatcgccagatacatcaggctgcaccccacccactacagcatcaggagcaccctgaggatggagctgatgggctgtgacctgaacagctgcagcatgcccctgggcatggagagcaaggccatctctgacgcccagatcactgcctccagctacttcaccaacatgtttgccacctggagccccagcaaggccaggctgcacctgcagggcaggagcaatgcctggaggccccaggtcaacaaccccaaggagtggctgcaggtggacttccagaagaccatgaaggtgactggggtgaccacccagggggtgaagagcctgctgaccagcatgtacgtgaaggagttcctgatctccagcagccaggacggccaccagtggaccctgttcttccagaatggcaaggtgaaggtgttccagggcaaccaggacagcttcacccctgtggtcaacagcctggacccccccctgctgaccagatacctgaggatccacccccagagctgggtgcaccagatcgccctgaggatggaggtgctgggctgtgaggcccaggacctgtactga

SEQ ID NO: 5 - DNA, 4374 bp, Artificial Sequence
  coFVIII-25
atgcagattgagctgagcacctgcttcttcctgtgcctgctgaggttctgcttctctgccaccaggagatactacctgggcgccgtggagctgagctgggactacatgcagtctgacctgggcgagctgccagtggacgccaggttcccccccagagtgcccaagagcttccccttcaacaccagcgtggtgtacaagaagaccctgttcgtggagttcactgaccacctgttcaacatcgccaagcccaggcccccctggatgggcctgctgggccccaccatccaggccgaggtgtacgacaccgtggtcatcaccctgaagaacatggccagccaccccgtctccctgcacgccgtgggggtgagctactggaaggcctctgagggcgccgagtacgacgaccagaccagccagagggagaaggaggacgacaaggtgttccctgggggcagccacacctacgtgtggcaggtcctgaaggagaacggccccatggcctctgaccccctgtgcctgacctacagctacctgagccacgtggacctggtgaaggacctgaactctggcctgattggggccctgctggtgtgcagggagggcagcctggccaaggagaagacccagaccctgcacaagttcatcctgctgttcgccgtgttcgacgagggcaagagctggcactctgaaaccaagaacagcctgatgcaggacagggacgccgcctctgccagggcctggcccaagatgcacaccgtcaacggctacgtcaacaggagcctgcctggcctgattggctgccacaggaagagcgtgtactggcatgtgatcggcatgggcaccacccctgaggtgcacagcatcttcctggagggccacaccttcctggtcaggaaccacaggcaggccagcctggagatcagccccatcaccttcctgaccgcccagaccctgctgatggacctgggccagttcctgctgttctgccacatctccagccaccagcacgacggcatggaggcctacgtgaaagtggacagctgccctgaggagccccagctgaggatgaagaacaacgaggaggccgaggactatgatgacgacctgaccgacagcgagatggacgtggtcaggttcgacgacgacaacagccccagcttcatccagatcaggagcgtggccaagaagcaccccaagacctgggtgcactacatcgctgctgaggaggaggactgggactatgcccccctggtgctggcccctgatgacaggagctacaagagccagtacctgaacaatggcccccagaggattggcaggaagtacaagaaagtcaggttcatggcctacactgatgaaaccttcaagaccagggaggccatccagcatgagtctggcatcctgggccccctgctgtacggggaggtgggggacaccctgctgatcatcttcaagaaccaggccagcaggccctacaacatctacccccatggcatcaccgacgtgaggcccctgtacagcaggaggctgcctaagggggtgaagcacctgaaagacttccccatcctgcctggggagatcttcaagtacaagtggactgtgactgtggaggacggccccaccaagagcgaccccaggtgcctgaccagatactacagcagcttcgtcaacatggagagggacctggcctctggcctgattggccccctgctgatctgctacaaggagtctgtggaccagaggggcaaccagatcatgagcgacaagaggaacgtgatcctgttctctgtcttcgacgagaacaggagctggtacctgactgaaaacatccagcggttcctccccaaccccgcgggcgtgcagctggaagatcctgagtttcaggcatcaaacatcatgcactccattaacggctacgtgttcgattcgctgcagctgagcgtgtgtctgcacgaagtggcctactggtacatcctgtccattggtgcccagactgacttcctgtccgtgtttttctccggctacacgttcaagcacaagatggtgtacgaggacaccctgaccctcttccctttttccggcgaaactgtgtttatgagcatggagaatcccggcctgtggatcttgggctgccacaacagcgacttccgtaacagaggaatgactgcgctgctcaaggtgtccagctgcgacaagaacaccggagactattatgaggactcatacgaggacatctccgcctacctcctgtccaagaataacgccattgaacctcggagcttcagccagaacccacccgtgcttaagagacatcaacgggagatcactaggaccaccctgcagtcagaccaggaggaaatcgactacgatgacaccatctcggtcgagatgaagaaggaggactttgacatctacgacgaagatgaaaaccagagcccgaggtcgttccaaaagaaaacccgccactactttattgctgctgtcgagcggctgtgggactacggaatgtcgtcctcgccgcacgtgctccgcaaccgagcccagagcggctcggtgccgcaattcaagaaggtcgtgttccaggagttcactgacgggagcttcactcagcctttgtaccggggagaactcaatgaacatctcggcctcctcggaccttacatcagagcagaagtggaagataacatcatggtcactttccgtaaccaagccagccgcccgtactcgttctactcctccctcatttcttacgaagaggaccagcggcagggcgcagaaccgcgcaagaacttcgtgaagcccaacgaaaccaagacctacttctggaaagtgcagcatcatatggccccgactaaggacgagtttgactgcaaagcctgggcctacttctccgatgtggacttggagaaggacgtccactccggcctcatcggtcccctgctcgtgtgccataccaataccctgaaccccgcacacggtcgccaggtcaccgtgcaggagttcgctctgttcttcactatcttcgacgaaactaagtcctggtacttcaccgagaacatggagaggaactgcagagccccctgtaacatccagatggaggacccgacgttcaaggaaaactaccggttccacgccattaacggatacatcatggatacgctgccgggtcttgtgatggcccaggatcaacggatcagatggtacttattgtcgatgggcagcaacgagaacatccactctattcacttctccggtcatgtgttcactgtgcggaagaaggaagagtacaagatggccctgtacaacctttatcccggagtgttcgaaactgtggaaatgctgccgtcgaaggccggcatttggcgcgtggagtgtttgattggagaacatctccatgcggggatgtcaaccctgttcctggtgtatagcaacaagtgccagactccgcttgggatggcgtcaggacacattagggatttccagatcactgcgtccggccagtacggccaatgggcccctaagctggcccgcctgcattactccggatccattaacgcctggtcaaccaaggagccattctcctggatcaaggtggaccttctggcccccatgattatccacggaattaagacccagggggcccggcagaagttctcctcactgtacatcagccagttcataatcatgtactccctggacggaaagaagtggcaaacctacagggggaacagcaccggcacactgatggtctttttcggaaatgtggactcctccgggattaagcataacatcttcaaccctccgattatcgctcggtacattagacttcaccctacccactacagcattcgctccaccctgcggatggaactgatgggctgcgatctgaactcgtgcagcatgccgttgggaatggagtccaaagcaatttccgacgcgcagatcaccgcctcgtcctactttaccaacatgttcgccacgtggtcaccgtccaaggcccggctgcacctccagggaagatccaacgcatggcggccacaggtcaacaaccctaaggagtggctccaggtggacttccagaaaaccatgaaggtcaccggagtcacaacccagggagtgaagtcgctgctgacttctatgtacgtcaaggagttcctgatctccagcagccaggacgggcaccagtggaccctgttcttccaaaatggaaaggtcaaggtgtttcagggcaatcaggattcattcaccccggtggtgaactcccttgatccacccctcctgacccgctaccttcgcatccacccacagtcctgggtgcaccagatcgcgctgaggatggaggtcctgggatgcgaagcccaggacctgtactga

SEQ ID NO: 6 - DNA, 4374 bp, Artificial Sequence
  coFVIII-26
atgcagattgagctgagcacctgcttcttcctgtgcctgctgaggttctgcttctctgccaccaggagatactacctgggcgccgtggagctgagctgggactacatgcagtctgacctgggcgagctgccagtggacgccaggttcccccccagagtgcccaagagcttccccttcaacaccagcgtggtgtacaagaagaccctgttcgtggagttcactgaccacctgttcaacatcgccaagcccaggcccccctggatgggcctgctgggccccaccatccaggccgaggtgtacgacaccgtggtcatcaccctgaagaacatggccagccaccccgtctccctgcacgccgtgggggtgagctactggaaggcctctgagggcgccgagtacgacgaccagaccagccagagggagaaggaggacgacaaggtgttccctgggggcagccacacctacgtgtggcaggtcctgaaggagaacggccccatggcctctgaccccctgtgcctgacctacagctacctgagccacgtggacctggtgaaggacctgaactctggcctgattggggccctgctggtgtgcagggagggcagcctggccaaggagaagacccagaccctgcacaagttcatcctgctgttcgccgtgttcgacgagggcaagagctggcactctgaaaccaagaacagcctgatgcaggacagggacgccgcctctgccagggcctggcccaagatgcacaccgtcaacggctacgtcaacaggagcctgcctggcctgattggctgccacaggaagagcgtgtactggcatgtgatcggcatgggcaccacccctgaggtgcacagcatcttcctggagggccacaccttcctggtcaggaaccacaggcaggccagcctggagatcagccccatcaccttcctgaccgcccagaccctgctgatggacctgggccagttcctgctgttctgccacatctccagccaccagcacgacggcatggaggcctacgtgaaagtggacagctgccctgaggagccccagctgaggatgaagaacaacgaggaggccgaggactatgatgacgacctgaccgacagcgagatggacgtggtcaggttcgacgacgacaacagccccagcttcatccagatcaggagcgtggccaagaagcaccccaagacctgggtgcactacatcgctgctgaggaggaggactgggactatgcccccctggtgctggcccctgatgacaggagctacaagagccagtacctgaacaatggcccccagaggattggcaggaagtacaagaaagtcaggttcatggcctacactgatgaaaccttcaagaccagggaggccatccagcatgagtctggcatcctgggccccctgctgtacggggaggtgggggacaccctgctgatcatcttcaagaaccaggccagcaggccctacaacatctacccccatggcatcaccgacgtgaggcccctgtacagcaggaggctgcctaagggggtgaagcacctgaaagacttccccatcctgcctggggagatcttcaagtacaagtggactgtgactgtggaggacggccccaccaagagcgaccccaggtgcctgaccagatactacagcagcttcgtcaacatggagagggacctggcctctggcctgattggccccctgctgatctgctacaaggagtctgtggaccagaggggcaaccagatcatgagcgacaagaggaacgtgatcctgttctctgtcttcgacgagaacaggagctggtacctcactgaaaacatccagaggttcctcccaaaccccgcaggagtgcaactggaggaccctgagtttcaggcctcgaatatcatgcactcgattaacggttacgtgttcgactcgctgcagctgagcgtgtgcctccatgaagtcgcttactggtacattctgtccatcggcgcccagactgacttcctgagcgtgttcttttccggttacacctttaagcacaagatggtgtacgaagataccctgaccctgttccctttctccggcgaaacggtgttcatgtcgatggagaacccgggtctgtggattctgggatgccacaacagcgactttcggaaccgcggaatgactgccctgctgaaggtgtcctcatgcgacaagaacaccggagactactacgaggactcctacgaggatatctcagcctacctcctgtccaagaacaacgcgatcgagccgcgcagcttcagccagaacccgcctgtgctgaagaggcaccagcgagaaattacccggaccaccctccaatcggatcaggaggaaatcgactacgacgacaccatctcggtggaaatgaagaaggaagatttcgatatctacgacgaggacgaaaatcagtcccctcgctcattccaaaagaaaactagacactactttatcgccgcggtggaaagactgtgggactatggaatgtcatccagccctcacgtccttcggaaccgggcccagagcggatcggtgcctcagttcaagaaagtggtgttccaggagttcaccgacggcagcttcacccagccgctgtaccggggagaactgaacgaacacctgggcctgctcggtccctacatccgcgcggaagtggaggataacatcatggtgaccttccgtaaccaagcatccagaccttactccttctattcctccctgatctcatacgaggaggaccagcgccaaggcgccgagccccgcaagaacttcgtcaagcccaacgagactaagacctacttctggaaggtccaacaccatatggccccgaccaaggatgagtttgactgcaaggcctgggcctacttctccgacgtggaccttgagaaggatgtccattccggcctgatcgggccgctgctcgtgtgtcacaccaacaccctgaacccagcgcatggacgccaggtcaccgtccaggagtttgctctgttcttcaccatttttgacgaaactaagtcctggtacttcaccgagaatatggagcgaaactgtagagcgccctgcaatatccagatggaagatccgactttcaaggagaactatagattccacgccatcaacgggtacatcatggatactctgccggggctggtcatggcccaggatcagaggattcggtggtacttgctgtcaatgggatcgaacgaaaacattcactccattcacttctccggtcacgtgttcactgtgcgcaagaaggaggagtacaagatggcgctgtacaatctgtaccccggggtgttcgaaactgtggagatgctgccgtccaaggccggcatctggagagtggagtgcctgatcggagagcacctccacgcggggatgtccaccctcttcctggtgtactcgaataagtgccagaccccgctgggcatggcctcgggccacatcagagacttccagatcacagcaagcggacaatacggccaatgggcgccgaagctggcccgcttgcactactccggatcgatcaacgcatggtccaccaaggaaccgttctcgtggattaaggtggacctcctggcccctatgattatccacggaattaagacccagggcgccaggcagaagttctcctccctgtacatctcgcaattcatcatcatgtacagcctggacgggaagaagtggcagacttacaggggaaactccaccggcaccctgatggtctttttcggcaacgtggattcctccggcattaagcacaacatcttcaacccaccgatcatagccagatatattaggctccaccccactcactactcaatccgctcaactcttcggatggaactcatggggtgcgacctgaactcctgctccatgccgttggggatggaatcaaaggctattagcgacgcccagatcaccgcgagctcctacttcactaacatgttcgccacctggagcccctccaaggccaggctgcacttgcagggacggtcaaatgcctggcggccgcaagtgaacaatccgaaggaatggcttcaagtggatttccaaaagaccatgaaagtgaccggagtcaccacccagggagtgaagtcccttctgacctcgatgtatgtgaaggagttcctgattagcagcagccaggacgggcaccagtggaccctgttcttccaaaacggaaaggtcaaggtgttccaggggaaccaggactcgttcacacccgtggtgaactccctggaccccccactgctgacgcggtacttgaggattcatcctcagtcctgggtccatcagattgcattgcgaatggaagtcctgggctgcgaggcccaggacctgtactga

SEQ ID NO: 7 - DNA, 1734 bp, Artificial Sequence
  coFVIII-52-NT58
gcgacccgccgatactacctgggagcagtggagctctcctgggattacatgcagagcgaccttggggagctgcccgtggatgccaggttccctccccgggtgccaaagtcgtttccgttcaacacctccgtggtgtacaagaaaactctgttcgtggagttcaccgaccacctgttcaatatcgccaagcccagacctccctggatggggctgttgggacctaccatccaagcggaggtgtacgacactgtggtcatcactctgaagaacatggcctcgcatcccgtgtccctgcacgccgtgggagtgtcttactggaaagcgtccgagggggccgaatacgacgaccagacctcgcagagagaaaaggaagatgacaaggtgttcccaggaggatcgcacacctacgtgtggcaagtgttgaaggagaacggcccaatggcctccgacccgctgtgcctgacctactcgtacctgtcccacgtggacctcgtgaaggacctcaactcgggactgattggagccctgctggtctgcagggaaggctcactggcgaaagaaaagactcagaccttgcacaagttcattctgctgttcgctgtgttcgacgaggggaagtcgtggcacagcgagactaagaactccctgatgcaagatagagatgccgcctccgcccgggcctggcctaagatgcacaccgtgaacggttacgtgaaccgctccctccctggcctgattggatgccaccggaagtccgtgtactggcacgtgatcgggatggggaccacccccgaggtgcacagcatcttcctggaaggtcacacatttctcgtgcgcaaccaccggcaggcctccctggaaatcagccccattaccttcctcactgcccagactctgctgatggacctgggacagttcctgctgttctgccatatctcctcccaccaacatgacggaatggaggcatacgtgaaggtcgattcctgccctgaggaaccccagctccgcatgaagaacaatgaggaagccgaggactacgacgacgacctgacggatagcgagatggatgtggtccggttcgatgacgataacagcccttccttcatccaaattcgctcggtggcaaagaagcaccccaagacctgggtgcattacattgcggcggaagaagaggactgggattatgccccgcttgtcctcgctcctgacgaccggagctacaagagccagtacctgaacaacggtccacagaggatcggtagaaagtacaagaaggtccgcttcatggcctataccgacgaaaccttcaaaactagagaggccatccaacacgaatccggcatcctgggcccgctcttgtacggagaagtcggcgacacccttctcattatcttcaagaaccaggcttcccggccgtacaacatctatccgcatgggatcactgacgtgcgcccactgtactcgcggcgcctgcccaagggtgtcaaacacctgaaggattttccgatccttccgggagaaatcttcaagtacaagtggaccgtgaccgtggaagatggcccaactaagtctgaccctagatgcctcacccgctactactcatccttcgtcaacatggagcgcgacctggccagcggactgatcggcccgctgctgatttgctacaaggaatcagtggaccaacggggaaaccagatcatgtcggataagaggaacgtcatcctcttctccgtg

SEQ ID NO: 8 - DNA, 2583 bp, Artificial Sequence
  coFVIII-52-CT
tttgacgaaaaccggtcgtggtacctgaccgagaacatccagaggttcctgcccaaccctgctggggtgcagctggaggaccccgagttccaggccagcaacatcatgcacagcatcaatggctacgtgttcgacagcctgcagctgagcgtgtgcctgcacgaggtggcctactggtacatcctgagcatcggcgcccagaccgacttcctgagcgtgttcttctctggctacaccttcaagcacaagatggtgtatgaggacaccctgaccctgttccccttcagcggggagactgtcttcatgagcatggagaaccctggcctgtggatcctgggctgccacaacagcgacttcaggaacaggggcatgactgccctgctgaaagtctccagctgtgacaagaacaccggggactactacgaggacagctacgaggacatcagcgcctacctgctgagcaagaacaatgccatcgagcccaggagcttctctcagaaccccccagtgctgaagaggcaccagagggagatcaccaggaccaccctgcagtctgaccaggaggagatcgactatgatgacaccatcagcgtggagatgaagaaggaggacttcgacatctacgacgaggacgagaaccagagccccaggagcttccagaagaagaccaggcactacttcattgctgctgtggagaggctgtgggactatggcatgtccagcagcccccatgtgctgaggaacagggcccagtctggcagcgtgccccagttcaagaaagtcgtgttccaggagttcaccgacggcagcttcacccagcccctgtacagaggggagctgaacgagcacctgggcctgctgggcccctacatcagggccgaggtggaggacaacatcatggtgaccttcaggaaccaggccagcaggccctacagcttctacagcagcctgatcagctacgaggaggaccagaggcagggggctgagcccaggaagaactttgtgaagcccaatgaaaccaagacctacttctggaaggtgcagcaccacatggcccccaccaaggacgagttcgactgcaaggcctgggcctacttctctgacgtggacctggagaaggacgtgcactctggcctgattggccccctgctggtgtgccacaccaacaccctgaaccctgcccatggcaggcaggtgactgtgcaggagttcgccctgttcttcaccatcttcgatgaaaccaagagctggtacttcactgagaacatggagaggaactgcagggccccctgcaacatccagatggaggaccccaccttcaaggagaactacaggttccatgccatcaatggctacatcatggacaccctgcctggcctggtcatggcccaggaccagaggatcaggtggtatctgctgagcatgggcagcaacgagaacatccacagcatccacttctctggccacgtgttcactgtgaggaagaaggaggagtacaagatggccctgtacaacctgtaccctggggtgttcgaaaccgtggagatgctgcccagcaaggccggcatctggagggtggagtgcctgattggggagcacctgcacgccggcatgagcaccctgttcctggtgtacagcaacaagtgccagacccccctgggcatggcctctggccacatcagggacttccagatcactgcctctggccagtacggccagtgggcccccaagctggccaggctgcactactccggaagcatcaatgcctggagcaccaaggagcccttcagctggatcaaagtggacctgctggcccccatgatcatccacggcatcaagacccagggggccaggcagaagttctccagcctgtacatcagccagttcatcatcatgtacagcctggacggcaagaagtggcagacctacaggggcaacagcaccggcaccctgatggtgttcttcggcaacgtggacagcagcggcatcaagcacaacatcttcaacccccccatcatcgccagatacatcaggctgcaccccacccactacagcatcaggagcaccctgaggatggagctgatgggctgtgacctgaacagctgcagcatgcccctgggcatggagagcaaggccatctctgacgcccagatcactgcctccagctacttcaccaacatgtttgccacctggagccccagcaaggccaggctgcacctgcagggcaggagcaatgcctggaggccccaggtcaacaaccccaaggagtggctgcaggtggacttccagaagaccatgaaggtgactggggtgaccacccagggggtgaagagcctgctgaccagcatgtacgtgaaggagttcctgatctccagcagccaggacggccaccagtggaccctgttcttccagaatggcaaggtgaaggtgttccagggcaaccaggacagcttcacccctgtggtcaacagcctggacccccccctgctgaccagatacctgaggatccacccccagagctgggtgcaccagatcgccctgaggatggaggtgctgggctgtgaggcccaggacctgtactga

SEQ ID NO: 9 - DNA, 1734 bp, Artificial Sequence
  coFVIII-62-NT58
gccactcgccggtactaccttggagccgtggagctttcatgggactacatgcagagcgacctgggcgaactccccgtggatgccagattccccccccgcgtgccaaagtccttcccctttaacacctccgtggtgtacaagaaaaccctctttgtcgagttcactgaccacctgttcaacatcgccaagccgcgcccaccttggatgggcctcctgggaccgaccattcaagctgaagtgtacgacaccgtggtgatcaccctgaagaacatggcgtcccaccccgtgtccctgcatgcggtcggagtgtcctactggaaggcctccgaaggagctgagtacgacgaccagactagccagcgggaaaaggaggacgataaagtgttcccgggcggctcgcatacttacgtgtggcaagtcctgaaggaaaacggacctatggcatccgatcctctgtgcctgacttactcctacctttcccatgtggacctcgtgaaggacctgaacagcgggctgattggtgcacttctcgtgtgccgcgaaggttcgctcgctaaggaaaagacccagaccctccataagttcatccttttgttcgctgtgttcgatgaaggaaagtcatggcattccgaaactaagaactcgctgatgcaggaccgggatgccgcctcagcccgcgcctggcctaaaatgcatacagtcaacggatacgtgaatcggtcactgcccgggctcatcggttgtcacagaaagtccgtgtactggcacgtcatcggcatgggcactacgcctgaagtgcactccatcttcctggaagggcacaccttcctcgtgcgcaaccaccgccaggcctctctggaaatctccccgattacctttctgaccgcccagactctgctcatggacctggggcagttccttctcttctgccacatctccagccatcagcacgacggaatggaggcctacgtgaaggtggactcatgcccggaagaacctcagttgcggatgaagaacaacgaggaggccgaggactatgacgacgatttgactgactccgagatggacgtcgtgcggttcgatgacgacaacagccccagcttcatccagattcgcagcgtggccaagaagcaccccaaaacctgggtgcactacatcgcggccgaggaagaagattgggactacgccccgttggtgctggcacccgatgaccggtcgtacaagtcccagtatctgaacaatggtccgcagcggattggcagaaagtacaagaaagtgcggttcatggcgtacactgacgaaacgtttaagacccgggaggccattcaacatgagagcggcattctgggaccactgctgtacggagaggtcggcgataccctgctcatcatcttcaaaaaccaggcctcccggccttacaacatctaccctcacggaatcaccgacgtgcggccactctactcgcggcgcctgccgaagggcgtcaagcacctgaaagacttccctatcctgccgggcgaaatcttcaagtataagtggaccgtcaccgtggaggacgggcccaccaagagcgatcctaggtgtctgactcggtactactccagcttcgtgaacatggaacgggacctggcatcgggactcattggaccgctgctgatctgctacaaagagtcggtggatcaacgcggcaaccagatcatgtccgacaagcgcaacgtgatcctgttctccgtg

SEQ ID NO: 10 - DNA, 2583 bp, Artificial Sequence
  coFVIII-62-CT
tttgatgaaaacagatcctggtacctgaccgagaacatccagaggttcctgcccaaccctgctggggtgcagctggaggaccccgagttccaggccagcaacatcatgcacagcatcaatggctacgtgttcgacagcctgcagctgagcgtgtgcctgcacgaggtggcctactggtacatcctgagcatcggcgcccagaccgacttcctgagcgtgttcttctctggctacaccttcaagcacaagatggtgtatgaggacaccctgaccctgttccccttcagcggggagactgtcttcatgagcatggagaaccctggcctgtggatcctgggctgccacaacagcgacttcaggaacaggggcatgactgccctgctgaaagtctccagctgtgacaagaacaccggggactactacgaggacagctacgaggacatcagcgcctacctgctgagcaagaacaatgccatcgagcccaggagcttctctcagaaccccccagtgctgaagaggcaccagagggagatcaccaggaccaccctgcagtctgaccaggaggagatcgactatgatgacaccatcagcgtggagatgaagaaggaggacttcgacatctacgacgaggacgagaaccagagccccaggagcttccagaagaagaccaggcactacttcattgctgctgtggagaggctgtgggactatggcatgtccagcagcccccatgtgctgaggaacagggcccagtctggcagcgtgccccagttcaagaaagtcgtgttccaggagttcaccgacggcagcttcacccagcccctgtacagaggggagctgaacgagcacctgggcctgctgggcccctacatcagggccgaggtggaggacaacatcatggtgaccttcaggaaccaggccagcaggccctacagcttctacagcagcctgatcagctacgaggaggaccagaggcagggggctgagcccaggaagaactttgtgaagcccaatgaaaccaagacctacttctggaaggtgcagcaccacatggcccccaccaaggacgagttcgactgcaaggcctgggcctacttctctgacgtggacctggagaaggacgtgcactctggcctgattggccccctgctggtgtgccacaccaacaccctgaaccctgcccatggcaggcaggtgactgtgcaggagttcgccctgttcttcaccatcttcgatgaaaccaagagctggtacttcactgagaacatggagaggaactgcagggccccctgcaacatccagatggaggaccccaccttcaaggagaactacaggttccatgccatcaatggctacatcatggacaccctgcctggcctggtcatggcccaggaccagaggatcaggtggtatctgctgagcatgggcagcaacgagaacatccacagcatccacttctctggccacgtgttcactgtgaggaagaaggaggagtacaagatggccctgtacaacctgtaccctggggtgttcgaaaccgtggagatgctgcccagcaaggccggcatctggagggtggagtgcctgattggggagcacctgcacgccggcatgagcaccctgttcctggtgtacagcaacaagtgccagacccccctgggcatggcctctggccacatcagggacttccagatcactgcctctggccagtacggccagtgggcccccaagctggccaggctgcactactccggaagcatcaatgcctggagcaccaaggagcccttcagctggatcaaagtggacctgctggcccccatgatcatccacggcatcaagacccagggggccaggcagaagttctccagcctgtacatcagccagttcatcatcatgtacagcctggacggcaagaagtggcagacctacaggggcaacagcaccggcaccctgatggtgttcttcggcaacgtggacagcagcggcatcaagcacaacatcttcaacccccccatcatcgccagatacatcaggctgcaccccacccactacagcatcaggagcaccctgaggatggagctgatgggctgtgacctgaacagctgcagcatgcccctgggcatggagagcaaggccatctctgacgcccagatcactgcctccagctacttcaccaacatgtttgccacctggagccccagcaaggccaggctgcacctgcagggcaggagcaatgcctggaggccccaggtcaacaaccccaaggagtggctgcaggtggacttccagaagaccatgaaggtgactggggtgaccacccagggggtgaagagcctgctgaccagcatgtacgtgaaggagttcctgatctccagcagccaggacggccaccagtggaccctgttcttccagaatggcaaggtgaaggtgttccagggcaaccaggacagcttcacccctgtggtcaacagcctggacccccccctgctgaccagatacctgaggatccacccccagagctgggtgcaccagatcgccctgaggatggaggtgctgggctgtgaggcccaggacctgtactga

SEQ ID NO: 11 - DNA, 1734 bp, Artificial Sequence
  coFVIII-25-NT58
gccaccaggagatactacctgggcgccgtggagctgagctgggactacatgcagtctgacctgggcgagctgccagtggacgccaggttcccccccagagtgcccaagagcttccccttcaacaccagcgtggtgtacaagaagaccctgttcgtggagttcactgaccacctgttcaacatcgccaagcccaggcccccctggatgggcctgctgggccccaccatccaggccgaggtgtacgacaccgtggtcatcaccctgaagaacatggccagccaccccgtctccctgcacgccgtgggggtgagctactggaaggcctctgagggcgccgagtacgacgaccagaccagccagagggagaaggaggacgacaaggtgttccctgggggcagccacacctacgtgtggcaggtcctgaaggagaacggccccatggcctctgaccccctgtgcctgacctacagctacctgagccacgtggacctggtgaaggacctgaactctggcctgattggggccctgctggtgtgcagggagggcagcctggccaaggagaagacccagaccctgcacaagttcatcctgctgttcgccgtgttcgacgagggcaagagctggcactctgaaaccaagaacagcctgatgcaggacagggacgccgcctctgccagggcctggcccaagatgcacaccgtcaacggctacgtcaacaggagcctgcctggcctgattggctgccacaggaagagcgtgtactggcatgtgatcggcatgggcaccacccctgaggtgcacagcatcttcctggagggccacaccttcctggtcaggaaccacaggcaggccagcctggagatcagccccatcaccttcctgaccgcccagaccctgctgatggacctgggccagttcctgctgttctgccacatctccagccaccagcacgacggcatggaggcctacgtgaaagtggacagctgccctgaggagccccagctgaggatgaagaacaacgaggaggccgaggactatgatgacgacctgaccgacagcgagatggacgtggtcaggttcgacgacgacaacagccccagcttcatccagatcaggagcgtggccaagaagcaccccaagacctgggtgcactacatcgctgctgaggaggaggactgggactatgcccccctggtgctggcccctgatgacaggagctacaagagccagtacctgaacaatggcccccagaggattggcaggaagtacaagaaagtcaggttcatggcctacactgatgaaaccttcaagaccagggaggccatccagcatgagtctggcatcctgggccccctgctgtacggggaggtgggggacaccctgctgatcatcttcaagaaccaggccagcaggccctacaacatctacccccatggcatcaccgacgtgaggcccctgtacagcaggaggctgcctaagggggtgaagcacctgaaagacttccccatcctgcctggggagatcttcaagtacaagtggactgtgactgtggaggacggccccaccaagagcgaccccaggtgcctgaccagatactacagcagcttcgtcaacatggagagggacctggcctctggcctgattggccccctgctgatctgctacaaggagtctgtggaccagaggggcaaccagatcatgagcgacaagaggaacgtgatcctgttctctgtc

SEQ ID NO: 12 - DNA, 2583 bp, Artificial Sequence
  coFVIII-25-CT
ttcgacgagaacaggagctggtacctgactgaaaacatccagcggttcctccccaaccccgcgggcgtgcagctggaagatcctgagtttcaggcatcaaacatcatgcactccattaacggctacgtgttcgattcgctgcagctgagcgtgtgtctgcacgaagtggcctactggtacatcctgtccattggtgcccagactgacttcctgtccgtgtttttctccggctacacgttcaagcacaagatggtgtacgaggacaccctgaccctcttccctttttccggcgaaactgtgtttatgagcatggagaatcccggcctgtggatcttgggctgccacaacagcgacttccgtaacagaggaatgactgcgctgctcaaggtgtccagctgcgacaagaacaccggagactattatgaggactcatacgaggacatctccgcctacctcctgtccaagaataacgccattgaacctcggagcttcagccagaacccacccgtgcttaagagacatcaacgggagatcactaggaccaccctgcagtcagaccaggaggaaatcgactacgatgacaccatctcggtcgagatgaagaaggaggactttgacatctacgacgaagatgaaaaccagagcccgaggtcgttccaaaagaaaacccgccactactttattgctgctgtcgagcggctgtgggactacggaatgtcgtcctcgccgcacgtgctccgcaaccgagcccagagcggctcggtgccgcaattcaagaaggtcgtgttccaggagttcactgacgggagcttcactcagcctttgtaccggggagaactcaatgaacatctcggcctcctcggaccttacatcagagcagaagtggaagataacatcatggtcactttccgtaaccaagccagccgcccgtactcgttctactcctccctcatttcttacgaagaggaccagcggcagggcgcagaaccgcgcaagaacttcgtgaagcccaacgaaaccaagacctacttctggaaagtgcagcatcatatggccccgactaaggacgagtttgactgcaaagcctgggcctacttctccgatgtggacttggagaaggacgtccactccggcctcatcggtcccctgctcgtgtgccataccaataccctgaaccccgcacacggtcgccaggtcaccgtgcaggagttcgctctgttcttcactatcttcgacgaaactaagtcctggtacttcaccgagaacatggagaggaactgcagagccccctgtaacatccagatggaggacccgacgttcaaggaaaactaccggttccacgccattaacggatacatcatggatacgctgccgggtcttgtgatggcccaggatcaacggatcagatggtacttattgtcgatgggcagcaacgagaacatccactctattcacttctccggtcatgtgttcactgtgcggaagaaggaagagtacaagatggccctgtacaacctttatcccggagtgttcgaaactgtggaaatgctgccgtcgaaggccggcatttggcgcgtggagtgtttgattggagaacatctccatgcggggatgtcaaccctgttcctggtgtatagcaacaagtgccagactccgcttgggatggcgtcaggacacattagggatttccagatcactgcgtccggccagtacggccaatgggcccctaagctggcccgcctgcattactccggatccattaacgcctggtcaaccaaggagccattctcctggatcaaggtggaccttctggcccccatgattatccacggaattaagacccagggggcccggcagaagttctcctcactgtacatcagccagttcataatcatgtactccctggacggaaagaagtggcaaacctacagggggaacagcaccggcacactgatggtctttttcggaaatgtggactcctccgggattaagcataacatcttcaaccctccgattatcgctcggtacattagacttcaccctacccactacagcattcgctccaccctgcggatggaactgatgggctgcgatctgaactcgtgcagcatgccgttgggaatggagtccaaagcaatttccgacgcgcagatcaccgcctcgtcctactttaccaacatgttcgccacgtggtcaccgtccaaggcccggctgcacctccagggaagatccaacgcatggcggccacaggtcaacaaccctaaggagtggctccaggtggacttccagaaaaccatgaaggtcaccggagtcacaacccagggagtgaagtcgctgctgacttctatgtacgtcaaggagttcctgatctccagcagccaggacgggcaccagtggaccctgttcttccaaaatggaaaggtcaaggtgtttcagggcaatcaggattcattcaccccggtggtgaactcccttgatccacccctcctgacccgctaccttcgcatccacccacagtcctgggtgcaccagatcgcgctgaggatggaggtcctgggatgcgaagcccaggacctgtactga

SEQ ID NO: 13 - DNA, 1734 bp, Artificial Sequence; identical to SEQ ID NO: 11
  coFVIII-26-NT58

SEQ ID NO: 14 - DNA, 2583 bp, Artificial Sequence
  coFVIII-26-CT
ttcgacgagaacaggagctggtacctcactgaaaacatccagaggttcctcccaaaccccgcaggagtgcaactggaggaccctgagtttcaggcctcgaatatcatgcactcgattaacggttacgtgttcgactcgctgcagctgagcgtgtgcctccatgaagtcgcttactggtacattctgtccatcggcgcccagactgacttcctgagcgtgttcttttccggttacacctttaagcacaagatggtgtacgaagataccctgaccctgttccctttctccggcgaaacggtgttcatgtcgatggagaacccgggtctgtggattctgggatgccacaacagcgactttcggaaccgcggaatgactgccctgctgaaggtgtcctcatgcgacaagaacaccggagactactacgaggactcctacgaggatatctcagcctacctcctgtccaagaacaacgcgatcgagccgcgcagcttcagccagaacccgcctgtgctgaagaggcaccagcgagaaattacccggaccaccctccaatcggatcaggaggaaatcgactacgacgacaccatctcggtggaaatgaagaaggaagatttcgatatctacgacgaggacgaaaatcagtcccctcgctcattccaaaagaaaactagacactactttatcgccgcggtggaaagactgtgggactatggaatgtcatccagccctcacgtccttcggaaccgggcccagagcggatcggtgcctcagttcaagaaagtggtgttccaggagttcaccgacggcagcttcacccagccgctgtaccggggagaactgaacgaacacctgggcctgctcggtccctacatccgcgcggaagtggaggataacatcatggtgaccttccgtaaccaagcatccagaccttactccttctattcctccctgatctcatacgaggaggaccagcgccaaggcgccgagccccgcaagaacttcgtcaagcccaacgagactaagacctacttctggaaggtccaacaccatatggccccgaccaaggatgagtttgactgcaaggcctgggcctacttctccgacgtggaccttgagaaggatgtccattccggcctgatcgggccgctgctcgtgtgtcacaccaacaccctgaacccagcgcatggacgccaggtcaccgtccaggagtttgctctgttcttcaccatttttgacgaaactaagtcctggtacttcaccgagaatatggagcgaaactgtagagcgccctgcaatatccagatggaagatccgactttcaaggagaactatagattccacgccatcaacgggtacatcatggatactctgccggggctggtcatggcccaggatcagaggattcggtggtacttgctgtcaatgggatcgaacgaaaacattcactccattcacttctccggtcacgtgttcactgtgcgcaagaaggaggagtacaagatggcgctgtacaatctgtaccccggggtgttcgaaactgtggagatgctgccgtccaaggccggcatctggagagtggagtgcctgatcggagagcacctccacgcggggatgtccaccctcttcctggtgtactcgaataagtgccagaccccgctgggcatggcctcgggccacatcagagacttccagatcacagcaagcggacaatacggccaatgggcgccgaagctggcccgcttgcactactccggatcgatcaacgcatggtccaccaaggaaccgttctcgtggattaaggtggacctcctggcccctatgattatccacggaattaagacccagggcgccaggcagaagttctcctccctgtacatctcgcaattcatcatcatgtacagcctggacgggaagaagtggcagacttacaggggaaactccaccggcaccctgatggtctttttcggcaacgtggattcctccggcattaagcacaacatcttcaacccaccgatcatagccagatatattaggctccaccccactcactactcaatccgctcaactcttcggatggaactcatggggtgcgacctgaactcctgctccatgccgttggggatggaatcaaaggctattagcgacgcccagatcaccgcgagctcctacttcactaacatgttcgccacctggagcccctccaaggccaggctgcacttgcagggacggtcaaatgcctggcggccgcaagtgaacaatccgaaggaatggcttcaagtggatttccaaaagaccatgaaagtgaccggagtcaccacccagggagtgaagtcccttctgacctcgatgtatgtgaaggagttcctgattagcagcagccaggacgggcaccagtggaccctgttcttccaaaacggaaaggtcaaggtgttccaggggaaccaggactcgttcacacccgtggtgaactccctggaccccccactgctgacgcggtacttgaggattcatcctcagtcctgggtccatcagattgcattgcgaatggaagtcctgggctgcgaggcccaggacctgtactga

SEQ ID NO: 15 - protein, 2332 aa, Homo sapiens
ATRRYYLGAVELSWDYMQSDLGELPVDARFPPRVPKSFPFNTSVVYKKTLFVEFTDHLFNIAKPRPPWMGLLGPTIQAEVYDTVVITLKNMASHPVSLHAVGVSYWKASEGAEYDDQTSQREKEDDKVFPGGSHTYVWQVLKENGPMASDPLCLTYSYLSHVDLVKDLNSGLIGALLVCREGSLAKEKTQTLHKFILLFAVFDEGKSWHSETKNSLMQDRDAASARAWPKMHTVNGYVNRSLPGLIGCHRKSVYWHVIGMGTTPEVHSIFLEGHTFLVRNHRQASLEISPITFLTAQTLLMDLGQFLLFCHISSHQHDGMEAYVKVDSCPEEPQLRMKNNEEAEDYDDDLTDSEMDVVRFDDDNSPSFIQIRSVAKKHPKTWVHYIAAEEEDWDYAPLVLAPDDRSYKSQYLNNGPQRIGRKYKKVRFMAYTDETFKTREAIQHESGILGPLLYGEVGDTLLIIFKNQASRPYNIYPHGITDVRPLYSRRLPKGVKHLKDFPILPGEIFKYKWTVTVEDGPTKSDPRCLTRYYSSFVNMERDLASGLIGPLLICYKESVDQRGNQIMSDKRNVILFSVFDENRSWYLTENIQRFLPNPAGVQLEDPEFQASNIMHSINGYVFDSLQLSVCLHEVAYWYILSIGAQTDFLSVFFSGYTFKHKMVYEDTLTLFPFSGETVFMSMENPGLWILGCHNSDFRNRGMTALLKVSSCDKNTGDYYEDSYEDISAYLLSKNNAIEPRSFSQNSRHPSTRQKQFNATTIPENDIEKTDPWFAHRTPMPKIQNVSSSDLLMLLRQSPTPHGLSLSDLQEAKYETFSDDPSPGAIDSNNSLSEMTHFRPQLHHSGDMVFTPESGLQLRLNEKLGTTAATELKKLDFKVSSTSNNLISTIPSDNLAAGTDNTSSLGPPSMPVHYDSQLDTTLFGKKSSPLTESGGPLSLSEENNDSKLLESGLMNSQESSWGKNVSSTESGRLFKGKRAHGPALLTKDNALFKVSISLLKTNKTSNNSATNRKTHIDGPSLLIENSPSVWQNILESDTEFKKVTPLIHDRMLMDKNATALRLNHMSNKTTSSKNMEMVQQKKEGPIPPDAQNPDMSFFKMLFLPESARWIQRTHGKNSLNSGQGPSPKQLVSLGPEKSVEGQNFLSEKNKVVVGKGEFTKDVGLKEMVFPSSRNLFLTNLDNLHENNTHNQEKKIQEEIEKKETLIQENVVLPQIHTVTGTKNFMKNLFLLSTRQNVEGSYDGAYAPVLQDFRSLNDSTNRTKKHTAHFSKKGEEENLEGLGNQTKQIVEKYACTTRISPNTSQQNFVTQRSKRALKQFRLPLEETELEKRIIVDDTSTQWSKNMKHLTPSTLTQIDYNEKEKGAITQSPLSDCLTRSHSIPQANRSPLPIAKVSSFPSIRPIYLTRVLFQDNSSHLPAASYRKKDSGVQESSHFLQGAKKNNLSLAILTLEMTGDQREVGSLGTSATNSVTYKKVENTVLPKPDLPKTSGKVELLPKVHIYQKDLFPTETSNGSPGHLDLVEGSLLQGTEGAIKWNEANRPGKVPFLRVATESSAKTPSKLLDPLAWDNHYGTQIPKEEWKSQEKSPEKTAFKKKDTILSLNACESNHAIAAINEGQNKPEIEVTWAKQGRTERLCSQNPPVLKRHQREITRTTLQSDQEEIDYDDTISVEMKKEDFDIYDEDENQSPRSFQKKTRHYFIAAVERLWDYGMSSSPHVLRNRAQSGSVPQFKKVVFQEFTDGSFTQPLYRGELNEHLGLLGPYIRAEVEDNIMVTFRNQASRPYSFYSSLISYEEDQRQGAEPRKNFVKPNETKTYFWKVQHHMAPTKDEFDCKAWAYFSDVDLEKDVHSGLIGPLLVCHTNTLNPAHGRQVTVQEFALFFTIFDETKSWYFTENMERNCRAPCNIQMEDPTFKENYRFHAINGYIMDTLPGLVMAQDQRIRWYLLSMGSNENIHSIHFSGHVFTVRKKEEYKMALYNLYPGVFETVEMLPSKAGIWRVECLIGEHLHAGMSTLFLVYSNKCQTPLGMASGHIRDFQITASGQYGQWAPKLARLHYSGSINAWSTKEPFSWIKVDLLAPMIIHGIKTQGARQKFSSLYISQFIIMYSLDGKKWQTYRGNSTGTLMVFFGNVDSSGIKHNIFNPPIIARYIRLHPTHYSIRSTLRMELMGCDLNSCSMPLGMESKAISDAQITASSYFTNMFATWSPSKARLHLQGRSNAWRPQVNNPKEWLQVDFQKTMKVTGVTTQGVKSLLTSMYVKEFLISSSQDGHQWTLFFQNGKVKVFQGNQDSFTPVVNSLDPPLLTRYLRIHPQSWVHQIALRMEVLGCEAQDLY

SEQ ID NO: 16 - DNA, 4371 bp, Artificial Sequence
  BDD-FVIII (non-optimized; "parental"), Nucleotide Sequence
atgcaaatagagctctccacctgcttctttctgtgccttttgcgattctgctttagtgccaccagaagatactacctgggtgcagtggaactgtcatgggactatatgcaaagtgatctcggtgagctgcctgtggacgcaagatttcctcctagagtgccaaaatcttttccattcaacacctcagtcgtgtacaaaaagactctgtttgtagaattcacggatcaccttttcaacatcgctaagccaaggccaccctggatgggtctgctaggtcctaccatccaggctgaggtttatgatacagtggtcattacacttaagaacatggcttcccatcctgtcagtcttcatgctgttggtgtatcctactggaaagcttctgagggagctgaatatgatgatcagaccagtcaaagggagaaagaagatgataaagtcttccctggtggaagccatacatatgtctggcaggtcctgaaagagaatggtccaatggcctctgacccactgtgccttacctactcatatctttctcatgtggacctggtaaaagacttgaattcaggcctcattggagccctactagtatgtagagaagggagtctggccaaggaaaagacacagaccttgcacaaatttatactactttttgctgtatttgatgaagggaaaagttggcactcagaaacaaagaactccttgatgcaggatagggatgctgcatctgctcgggcctggcctaaaatgcacacagtcaatggttatgtaaacaggtctctgccaggtctgattggatgccacaggaaatcagtctattggcatgtgattggaatgggcaccactcctgaagtgcactcaatattcctcgaaggtcacacatttcttgtgaggaaccatcgccaggcgtccttggaaatctcgccaataactttccttactgctcaaacactcttgatggaccttggacagtttctactgttttgtcatatctcttcccaccaacatgatggcatggaagcttatgtcaaagtagacagctgtccagaggaaccccaactacgaatgaaaaataatgaagaagcggaagactatgatgatgatcttactgattctgaaatggatgtggtcaggtttgatgatgacaactctccttcctttatccaaattcgctcagttgccaagaagcatcctaaaacttgggtacattacattgctgctgaagaggaggactgggactatgctcccttagtcctcgcccccgatgacagaagttataaaagtcaatatttgaacaatggccctcagcggattggtaggaagtacaaaaaagtccgatttatggcatacacagatgaaacctttaagactcgtgaagctattcagcatgaatcaggaatcttgggacctttactttatggggaagttggagacacactgttgattatatttaagaatcaagcaagcagaccatataacatctaccctcacggaatcactgatgtccgtcctttgtattcaaggagattaccaaaaggtgtaaaacatttgaaggattttccaattctgccaggagaaatattcaaatataaatggacagtgactgtagaagatgggccaactaaatcagatcctcggtgcctgacccgctattactctagtttcgttaatatggagagagatctagcttcaggactcattggccctctcctcatctgctacaaagaatctgtagatcaaagaggaaaccagataatgtcagacaagaggaatgtcatcctgttttctgtatttgatgagaaccgaagctggtacctcacagagaatatacaacgctttctccccaatccagctggagtgcagcttgaggatccagagttccaagcctccaacatcatgcacagcatcaatggctatgtttttgatagtttgcagttgtcagtttgtttgcatgaggtggcatactggtacattctaagcattggagcacagactgacttcctttctgtcttcttctctggatataccttcaaacacaaaatggtctatgaagacacactcaccctattcccattctcaggagaaactgtcttcatgtcgatggaaaacccaggtctatggattctggggtgccacaactcagactttcggaacagaggcatgaccgccttactgaaggtttctagttgtgacaagaacactggtgattattacgaggacagttatgaagatatttcagcatacttgctgagtaaaaacaatgccattgaaccaagaagcttctctcaaaacccaccagtcttgaaacgccatcaacgggaaataactcgtactactcttcagtcagatcaagaggaaattgactatgatgataccatatcagttgaaatgaagaaggaagattttgacatttatgatgaggatgaaaatcagagcccccgcagctttcaaaagaaaacacgacactattttattgctgcagtggagaggctctgggattatgggatgagtagctccccacatgttctaagaaacagggctcagagtggcagtgtccctcagttcaagaaagttgttttccaggaatttactgatggctcctttactcagcccttataccgtggagaactaaatgaacatttgggactcctggggccatatataagagcagaagttgaagataatatcatggtaactttcagaaatcaggcctctcgtccctattccttctattctagccttatttcttatgaggaagatcagaggcaaggagcagaacctagaaaaaactttgtcaagcctaatgaaaccaaaacttacttttggaaagtgcaacatcatatggcacccactaaagatgagtttgactgcaaagcctgggcttatttctctgatgttgacctggaaaaagatgtgcactcaggcctgattggaccccttctggtctgccacactaacacactgaaccctgctcatgggagacaagtgacagtacaggaatttgctctgtttttcaccatctttgatgagaccaaaagctggtacttcactgaaaatatggaaagaaactgcagggctccctgcaatatccagatggaagatcccacttttaaagagaattatcgcttccatgcaatcaatggctacataatggatacactacctggcttagtaatggctcaggatcaaaggattcgatggtatctgctcagcatgggcagcaatgaaaacatccattctattcatttcagtggacatgtgttcactgtacgaaaaaaagaggagtataaaatggcactgtacaatctctatccaggtgtttttgagacagtggaaatgttaccatccaaagctggaatttggcgggtggaatgccttattggcgagcatctacatgctgggatgagcacactttttctggtgtacagcaataagtgtcagactcccctgggaatggcttctggacacattagagattttcagattacagcttcaggacaatatggacagtgggccccaaagctggccagacttcattattccggatcaatcaatgcctggagcaccaaggagcccttttcttggatcaaggtggatctgttggcaccaatgattattcacggcatcaagacccagggtgcccgtcagaagttctccagcctctacatctctcagtttatcatcatgtatagtcttgatgggaagaagtggcagacttatcgaggaaattccactggaaccttaatggtcttctttggcaatgtggattcatctgggataaaacacaatatttttaaccctccaattattgctcgatacatccgtttgcacccaactcattatagcattcgcagcactcttcgcatggagttgatgggctgtgatttaaatagttgcagcatgccattgggaatggagagtaaagcaatatcagatgcacagattactgcttcatcctactttaccaatatgtttgccacctggtctccttcaaaagctcgacttcacctccaagggaggagtaatgcctggagacctcaggtgaataatccaaaagagtggctgcaagtggacttccagaagacaatgaaagtcacaggagtaactactcagggagtaaaatctctgcttaccagcatgtatgtgaaggagttcctcatctccagcagtcaagatggccatcagtggactctcttttttcagaatggcaaagtaaaggtttttcagggaaatcaagactccttcacacctgtggtgaactctctagacccaccgttactgactcgctaccttcgaattcacccccagagttgggtgcaccagattgccctgaggatggaggttctgggctgcgaggcacaggacctctac

SEQ ID NO: 17 - protein, 1438 aa, Artificial Sequence
  BDD-FVIII (non-optimized; "parental"), Amino Acid Sequence
ATRRYYLGAVELSWDYMQSDLGELPVDARFPPRVPKSFPFNTSVVYKKTLFVEFTDHLFNIAKPRPPWMGLLGPTIQAEVYDTVVITLKNMASHPVSLHAVGVSYWKASEGAEYDDQTSQREKEDDKVFPGGSHTYVWQVLKENGPMASDPLCLTYSYLSHVDLVKDLNSGLIGALLVCREGSLAKEKTQTLHKFILLFAVFDEGKSWHSETKNSLMQDRDAASARAWPKMHTVNGYVNRSLPGLIGCHRKSVYWHVIGMGTTPEVHSIFLEGHTFLVRNHRQASLEISPITFLTAQTLLMDLGQFLLFCHISSHQHDGMEAYVKVDSCPEEPQLRMKNNEEAEDYDDDLTDSEMDVVRFDDDNSPSFIQIRSVAKKHPKTWVHYIAAEEEDWDYAPLVLAPDDRSYKSQYLNNGPQRIGRKYKKVRFMAYTDETFKTREAIQHESGILGPLLYGEVGDTLLIIFKNQASRPYNIYPHGITDVRPLYSRRLPKGVKHLKDFPILPGEIFKYKWTVTVEDGPTKSDPRCLTRYYSSFVNMERDLASGLIGPLLICYKESVDQRGNQIMSDKRNVILFSVFDENRSWYLTENIQRFLPNPAGVQLEDPEFQASNIMHSINGYVFDSLQLSVCLHEVAYWYILSIGAQTDFLSVFFSGYTFKHKMVYEDTLTLFPFSGETVFMSMENPGLWILGCHNSDFRNRGMTALLKVSSCDKNTGDYYEDSYEDISAYLLSKNNAIEPRSFSQNPPVLKRHQREITRTTLQSDQEEIDYDDTISVEMKKEDFDIYDEDENQSPRSFQKKTRHYFIAAVERLWDYGMSSSPHVLRNRAQSGSVPQFKKVVFQEFTDGSFTQPLYRGELNEHLGLLGPYIRAEVEDNIMVTFRNQASRPYSFYSSLISYEEDQRQGAEPRKNFVKPNETKTYFWKVQHHMAPTKDEFDCKAWAYFSDVDLEKDVHSGLIGPLLVCHTNTLNPAHGRQVTVQEFALFFTIFDETKSWYFTENMERNCRAPCNIQMEDPTFKENYRFHAINGYIMDTLPGLVMAQDQRIRWYLLSMGSNENIHSIHFSGHVFTVRKKEEYKMALYNLYPGVFETVEMLPSKAGIWRVECLIGEHLHAGMSTLFLVYSNKCQTPLGMASGHIRDFQITASGQYGQWAPKLARLHYSGSINAWSTKEPFSWIKVDLLAPMIIHGIKTQGARQKFSSLYISQFIIMYSLDGKKWQTYRGNSTGTLMVFFGNVDSSGIKHNIFNPPIIARYIRLHPTHYSIRSTLRMELMGCDLNSCSMPLGMESKAISDAQITASSYFTNMFATWSPSKARLHLQGRSNAWRPQVNNPKEWLQVDFQKTMKVTGVTTQGVKSLLTSMYVKEFLISSSQDGHQWTLFFQNGKVKVFQGNQDSFTPVVNSLDPPLLTRYLRIHPQSWVHQIALRMEVLGCEAQDLY

SEQ ID NO: 18 - DNA, 450 bp, Artificial Sequence
  XTEN nucleotide sequence
ggcgcgccaacatcagagagcgccacccctgaaagtggtcccgggagcgagccagccacatctgggtcggaaacgccaggcacaagtgagtctgcaactcccgagtccggacctggctccgagcctgccactagcggctccgagactccgggaacttccgagagcgctacaccagaaagcggacccggaaccagtaccgaacctagcgagggctctgctccgggcagcccagccggctctcctacatccacggaggagggcacttccgaatccgccaccccggagtcagggccaggatctgaacccgctacctcaggcagtgagacgccaggaacgagcgagtccgctacaccggagagtgggccagggagccctgctggatctcctacgtccactgaggaagggtcaccagcgggctcgcccaccagcactgaagaaggtgcctcgagc

SEQ ID NO: 19 - DNA, 4824 bp, Artificial Sequence
  coFVIII-52-XTEN
atgcaaatcgaactgagcacctgtttcttcctctgcctgctgagattctgtttctccgcgacccgccgatactacctgggagcagtggagctctcctgggattacatgcagagcgaccttggggagctgcccgtggatgccaggttccctccccgggtgccaaagtcgtttccgttcaacacctccgtggtgtacaagaaaactctgttcgtggagttcaccgaccacctgttcaatatcgccaagcccagacctccctggatggggctgttgggacctaccatccaagcggaggtgtacgacactgtggtcatcactctgaagaacatggcctcgcatcccgtgtccctgcacgccgtgggagtgtcttactggaaagcgtccgagggggccgaatacgacgaccagacctcgcagagagaaaaggaagatgacaaggtgttcccaggaggatcgcacacctacgtgtggcaagtgttgaaggagaacggcccaatggcctccgacccgctgtgcctgacctactcgtacctgtcccacgtggacctcgtgaaggacctcaactcgggactgattggagccctgctggtctgcagggaaggctcactggcgaaagaaaagactcagaccttgcacaagttcattctgctgttcgctgtgttcgacgaggggaagtcgtggcacagcgagactaagaactccctgatgcaagatagagatgccgcctccgcccgggcctggcctaagatgcacaccgtgaacggttacgtgaaccgctccctccctggcctgattggatgccaccggaagtccgtgtactggcacgtgatcgggatggggaccacccccgaggtgcacagcatcttcctggaaggtcacacatttctcgtgcgcaaccaccggcaggcctccctggaaatcagccccattaccttcctcactgcccagactctgctgatggacctgggacagttcctgctgttctgccatatctcctcccaccaacatgacggaatggaggcatacgtgaaggtcgattcctgccctgaggaaccccagctccgcatgaagaacaatgaggaagccgaggactacgacgacgacctgacggatagcgagatggatgtggtccggttcgatgacgataacagcccttccttcatccaaattcgctcggtggcaaagaagcaccccaagacctgggtgcattacattgcggcggaagaagaggactgggattatgccccgcttgtcctcgctcctgacgaccggagctacaagagccagtacctgaacaacggtccacagaggatcggtagaaagtacaagaaggtccgcttcatggcctataccgacgaaaccttcaaaactagagaggccatccaacacgaatccggcatcctgggcccgctcttgtacggagaagtcggcgacacccttctcattatcttcaagaaccaggcttcccggccgtacaacatctatccgcatgggatcactgacgtgcgcccactgtactcgcggcgcctgcccaagggtgtcaaacacctgaaggattttccgatccttccgggagaaatcttcaagtacaagtggaccgtgaccgtggaagatggcccaactaagtctgaccctagatgcctcacccgctactactcatccttcgtcaacatggagcgcgacctggccagcggactgatcggcccgctgctgatttgctacaaggaatcagtggaccaacggggaaaccagatcatgtcggataagaggaacgtcatcctcttctccgtgtttgacgaaaaccggtcgtggtacctgaccgagaacatccagaggttcctgcccaaccctgctggggtgcagctggaggaccccgagttccaggccagcaacatcatgcacagcatcaatggctacgtgttcgacagcctgcagctgagcgtgtgcctgcacgaggtggcctactggtacatcctgagcatcggcgcccagaccgacttcctgagcgtgttcttctctggctacaccttcaagcacaagatggtgtatgaggacaccctgaccctgttccccttcagcggggagactgtcttcatgagcatggagaaccctggcctgtggatcctgggctgccacaacagcgacttcaggaacaggggcatgactgccctgctgaaagtctccagctgtgacaagaacaccggggactactacgaggacagctacgaggacatcagcgcctacctgctgagcaagaacaatgccatcgagcccaggagcttctctcagaacggcgcgccaacatcagagagcgccacccctgaaagtggtcccgggagcgagccagccacatctgggtcggaaacgccaggcacaagtgagtctgcaactcccgagtccggacctggctccgagcctgccactagcggctccgagactccgggaacttccgagagcgctacaccagaaagcggacccggaaccagtaccgaacctagcgagggctctgctccgggcagcccagccggctctcctacatccacggaggagggcacttccgaatccgccaccccggagtcagggccaggatctgaacccgctacctcaggcagtgagacgccaggaacgagcgagtccgctacaccggagagtgggccagggagccctgctggatctcctacgtccactgaggaagggtcaccagcgggctcgcccaccagcactgaagaaggtgcctcgagccccccagtgctgaagaggcaccagagggagatcaccaggaccaccctgcagtctgaccaggaggagatcgactatgatgacaccatcagcgtggagatgaagaaggaggacttcgacatctacgacgaggacgagaaccagagccccaggagcttccagaagaagaccaggcactacttcattgctgctgtggagaggctgtgggactatggcatgtccagcagcccccatgtgctgaggaacagggcccagtctggcagcgtgccccagttcaagaaagtcgtgttccaggagttcaccgacggcagcttcacccagcccctgtacagaggggagctgaacgagcacctgggcctgctgggcccctacatcagggccgaggtggaggacaacatcatggtgaccttcaggaaccaggccagcaggccctacagcttctacagcagcctgatcagctacgaggaggaccagaggcagggggctgagcccaggaagaactttgtgaagcccaatgaaaccaagacctacttctggaaggtgcagcaccacatggcccccaccaaggacgagttcgactgcaaggcctgggcctacttctctgacgtggacctggagaaggacgtgcactctggcctgattggccccctgctggtgtgccacaccaacaccctgaaccctgcccatggcaggcaggtgactgtgcaggagttcgccctgttcttcaccatcttcgatgaaaccaagagctggtacttcactgagaacatggagaggaactgcagggccccctgcaacatccagatggaggaccccaccttcaaggagaactacaggttccatgccatcaatggctacatcatggacaccctgcctggcctggtcatggcccaggaccagaggatcaggtggtatctgctgagcatgggcagcaacgagaacatccacagcatccacttctctggccacgtgttcactgtgaggaagaaggaggagtacaagatggccctgtacaacctgtaccctggggtgttcgaaaccgtggagatgctgcccagcaaggccggcatctggagggtggagtgcctgattggggagcacctgcacgccggcatgagcaccctgttcctggtgtacagcaacaagtgccagacccccctgggcatggcctctggccacatcagggacttccagatcactgcctctggccagtacggccagtgggcccccaagctggccaggctgcactactccggaagcatcaatgcctggagcaccaaggagcccttcagctggatcaaagtggacctgctggcccccatgatcatccacggcatcaagacccagggggccaggcagaagttctccagcctgtacatcagccagttcatcatcatgtacagcctggacggcaagaagtggcagacctacaggggcaacagcaccggcaccctgatggtgttcttcggcaacgtggacagcagcggcatcaagcacaacatcttcaacccccccatcatcgccagatacatcaggctgcaccccacccactacagcatcaggagcaccctgaggatggagctgatgggctgtgacctgaacagctgcagcatgcccctgggcatggagagcaaggccatctctgacgcccagatcactgcctccagctacttcaccaacatgtttgccacctggagccccagcaaggccaggctgcacctgcagggcaggagcaatgcctggaggccccaggtcaacaaccccaaggagtggctgcaggtggacttccagaagaccatgaaggtgactggggtgaccacccagggggtgaagagcctgctgaccagcatgtacgtgaaggagttcctgatctccagcagccaggacggccaccagtggaccctgttcttccagaatggcaaggtgaaggtgttccagggcaaccaggacagcttcacccctgtggtcaacagcctggacccccccctgctgaccagatacctgaggatccacccccagagctgggtgcaccagatcgccctgaggatggaggtgctgggctgtgaggcccaggacctgtactga

SEQ ID NO: 20 - DNA, 4824 bp, Artificial Sequence
  coFVIII-1-XTEN
atgcagattgagctgtctacttgctttttcctgtgcctgctgaggttttgcttttccgctacacgaaggtattatctgggggctgtggaactgtcttgggattacatgcagagtgacctgggagagctgccagtggacgcaaggtttccccctagagtccctaagtcattccccttcaacactagcgtggtctacaagaaaacactgttcgtggagtttactgatcacctgttcaacatcgcaaagcctaggccaccctggatgggactgctggggccaacaatccaggccgaggtgtacgacaccgtggtcattacacttaagaacatggcctcacaccccgtgagcctgcatgctgtgggcgtcagctactggaaggcttccgaaggagcagagtatgacgatcagacttcccagagagaaaaagaggacgataaggtgtttcctggcggatctcatacctacgtgtggcaggtcctgaaagagaatggccctatggcctccgaccctctgtgcctgacctactcttatctgagtcacgtggacctggtcaaggatctgaacagcggcctgatcggagccctgctggtgtgcagggaaggaagcctggctaaggagaaaacccagacactgcataagttcattctgctgttcgccgtgtttgacgaagggaaatcatggcacagcgagacaaagaatagtctgatgcaggacagggatgccgcttcagccagagcttggcccaaaatgcacactgtgaacggctacgtcaatcgctcactgcctgggctgatcggctgccaccgaaagagcgtgtattggcatgtcatcgggatgggcaccacacctgaagtgcactccattttcctggagggacatacctttctggtccgcaaccaccgacaggcttccctggagatctctccaattaccttcctgacagcacagactctgctgatggacctggggcagttcctgctgttttgccacatcagctcccaccagcatgatggcatggaggcttacgtgaaagtggactcttgtcccgaggaacctcagctgcggatgaagaacaatgaggaagcagaagactatgacgatgacctgaccgactccgagatggatgtggtccgattcgatgacgataacagcccctcctttatccagattagatctgtggccaagaaacaccctaagacatgggtccattacatcgcagccgaggaagaggactgggattatgcaccactggtgctggcaccagacgatcgctcctacaaatctcagtatctgaacaatgggccacagaggattggcagaaagtacaagaaagtgcggttcatggcatataccgatgagaccttcaagactcgcgaagccatccagcacgagagcggcatcctgggaccactgctgtacggagaagtgggagacaccctgctgatcattttcaagaaccaggccagccggccttacaatatctatccacatgggattacagatgtgcgccctctgtacagcaggagactgccaaagggcgtcaaacacctgaaggacttcccaatcctgcccggagaaatcttcaagtacaagtggactgtcaccgtcgaggatggccccactaagagcgaccctcggtgcctgacccgctactattctagtttcgtgaatatggaaagagatctggcaagcggactgatcggaccactgctgatttgttacaaagagagcgtggatcagagaggcaaccagatcatgtccgacaagcggaatgtgattctgttcagtgtctttgacgaaaacaggtcatggtacctgaccgagaacatccagagattcctgcctaatccagctggggtgcagctggaagatcctgagtttcaggcatctaacatcatgcatagtattaatggctacgtgttcgacagtttgcagctgagcgtgtgcctgcacgaggtcgcttactggtatatcctgagcattggggcacagacagatttcctgagcgtgttcttttccggctacacttttaagcataaaatggtctatgaggacacactgactctgttccccttcagcggcgaaaccgtgtttatgagcatggagaatcccggactgtggattctggggtgccacaacagcgatttcagaaatcgcggaatgactgccctgctgaaagtgtcaagctgtgacaagaacaccggggactactatgaagattcatacgaggacatcagcgcatatctgctgtccaaaaacaatgccattgaaccccggtcttttagtcagaatggcgcgccaacatcagagagcgccacccctgaaagtggtcccgggagcgagccagccacatctgggtcggaaacgccaggcacaagtgagtctgcaactcccgagtccggacctggctccgagcctgccactagcggctccgagactccgggaacttccgagagcgctacaccagaaagcggacccggaaccagtaccgaacctagcgagggctctgctccgggcagcccagccggctctcctacatccacggaggagggcacttccgaatccgccaccccggagtcagggccaggatctgaacccgctacctcaggcagtgagacgccaggaacgagcgagtccgctacaccggagagtgggccagggagccctgctggatctcctacgtccactgaggaagggtcaccagcgggctcgcccaccagcactgaagaaggtgcctcgagccctccagtgctgaagcggcaccagcgcgagatcacccgcactaccctgcagagtgatcaggaagagatcgactacgacgatacaatttctgtggaaatgaagaaagaggacttcgatatctatgacgaagatgagaaccagagtcctcgatcattccagaagaaaaccaggcattactttattgccgcagtggagcggctgtgggattatggcatgtcctctagtcctcacgtgctgcgaaatagggcccagtcaggaagcgtcccacagttcaagaaagtggtcttccaggagtttacagacgggtcctttactcagccactgtacaggggcgaactgaacgagcacctgggactgctggggccctatatcagagcagaagtggaggataacattatggtcaccttcagaaatcaggcctctcggccttacagtttttattcaagcctgatctcttacgaagaggaccagcgacagggagctgaaccacgaaaaaacttcgtgaagcctaatgagaccaaaacatacttttggaaggtgcagcaccatatggccccaacaaaagacgagttcgattgcaaggcatgggcctatttttctgacgtggatctggagaaggacgtgcacagtggcctgattggcccactgctggtgtgccatactaacaccctgaatccagcccacggccggcaggtcactgtccaggagttcgctctgttctttaccatctttgatgagacaaagagctggtacttcaccgaaaacatggagcgaaattgcagggctccatgtaacattcagatggaagaccccacattcaaggagaactaccgctttcatgctatcaatggatacatcatggatactctgcccgggctggtcatggcacaggaccagagaatccggtggtatctgctgagcatgggcagcaacgagaatatccactcaattcatttcagcgggcacgtgtttactgtcaggaagaaagaagagtacaagatggccctgtacaacctgtatcccggcgtgttcgaaaccgtcgagatgctgcctagcaaggccggaatctggagagtggaatgcctgattggagagcacctgcatgctgggatgtctaccctgtttctggtgtacagtaataagtgtcagacacccctgggaatggcatccgggcatatcagggatttccagattaccgcatctggacagtacggacagtgggcacctaagctggctagactgcactattccggatctatcaacgcttggtccacaaaagagcctttctcttggattaaggtggacctgctggccccaatgatcattcatggcatcaaaactcagggagctcggcagaagttctcctctctgtacatctcacagtttatcatcatgtacagcctggatgggaagaaatggcagacataccgcggcaatagcacaggaactctgatggtgttctttggcaacgtggacagcagcggaatcaagcacaacattttcaatccccctatcattgctagatacatccggctgcacccaacccattattctattcgaagtacactgaggatggaactgatgggatgcgatctgaacagttgttcaatgcccctggggatggagtccaaggcaatctctgacgcccagattaccgccagctcctacttcactaatatgtttgctacctggagcccttccaaagcaagactgcacctgcaaggccgcagcaacgcatggcgaccacaggtgaacaatcccaaggagtggttgcaggtcgattttcagaaaactatgaaggtgaccggggtcacaactcagggcgtgaaaagtctgctgacctcaatgtacgtcaaggagttcctgatctctagttcacaggacggacatcagtggacactgttctttcagaacgggaaggtgaaagtcttccagggcaatcaggattcctttacacctgtggtcaacagtctagaccctccactgctgaccagatacctgagaatccaccctcagtcctgggtgcaccagattgccctgagaatggaagtgctgggatgcgaggcccaggatctgtactga

SEQ ID NO: 21 - DNA, 6 bp, Artificial Sequence
  MAR/ARS
atattt

SEQ ID NO: 22 - DNA, 6 bp, Artificial Sequence
  MAR/ARS
aaatat

SEQ ID NO: 23 - DNA, 5 bp, Artificial Sequence
  destabilizing element
attta

SEQ ID NO: 24 - DNA, 5 bp, Artificial Sequence
  destabilizing element
taaat

SEQ ID NO: 25 - DNA, 6 bp, Artificial Sequence
  poly-T site
tttttt

SEQ ID NO: 26 - DNA, 7 bp, Artificial Sequence
  poly-A site
aaaaaaa

SEQ ID NO: 27 - DNA, 6 bp, Artificial Sequence
  splice site
ggtgat

SEQ ID NO: 28 - DNA, 5 bp, Artificial Sequence
  TATA box
tataa

SEQ ID NO: 29 - DNA, 5 bp, Artificial Sequence
  TATA box
ttata

SEQ ID NO: 30 - DNA, 8 bp, Artificial Sequence
  AU rich sequence element
attttatt

SEQ ID NO: 31 - DNA, 8 bp, Artificial Sequence
  AU rich sequence element
atttttaa

SEQ ID NO: 32 - DNA, 13 bp, Artificial Sequence
  kozak consensus sequence
gccgccaccatgc

SEQ ID NO: 33 - protein, 32 aa, Artificial Sequence
  CTP peptide
DPRFQDSSSSKAPPPSLPSPSRLPGPSDTPIL

SEQ ID NO: 34 - protein, 28 aa, Artificial Sequence
  CTP peptide
SSSSKAPPPSLPSPSRLPGPSDTPILPQ

SEQ ID NO: 35 - protein, 11 aa, Artificial Sequence
  albumin-binding peptide core sequence
DICLPRWGCLW

SEQ ID NO: 36 - protein, 20 aa, Artificial Sequence
  PAS sequence
ASPAAPAPASPAAPAPSAPA

SEQ ID NO: 37 - protein, 20 aa, Artificial Sequence
  PAS sequence
AAPASPAPAAPSAPAPAAPS

SEQ ID NO: 38 - protein, 20 aa, Artificial Sequence
  PAS sequence
APSSPSPSAPSSPSPASPSS

SEQ ID NO: 39 - protein, 19 aa, Artificial Sequence
  PAS sequence
APSSPSPSAPSSPSPASPS

SEQ ID NO: 40 - protein, 20 aa, Artificial Sequence
  PAS sequence
SSPSAPSPSSPASPSPSSPA

SEQ ID NO: 41 - protein, 24 aa, Artificial Sequence
  PAS sequence
AASPAAPSAPPAAASPAAPSAPPA

SEQ ID NO: 42 - protein, 20 aa, Artificial Sequence
  PAS sequence
ASAAAPAAASAAASAPSAAA

SEQ ID NO: 43 - DNA, 23 bp, Artificial Sequence
  miR142 target
tccataaagtaggaaacactaca

SEQ ID NO: 44 - protein, 2332 aa, Homo sapiens; identical to SEQ ID NO: 15

SEQ ID NO: 45 - protein, 4 aa, Artificial Sequence
  amino acids 233-236 of human IgG1
ELLG

SEQ ID NO: 46 - protein, 42 aa, Artificial Sequence
  XTEN AE42-4, protein sequence
GAPGSPAGSPTSTEEGTSESATPESGPGSEPATSGSETPASS

SEQ ID NO: 47 - DNA, 126 bp, Artificial Sequence
  XTEN AE42-4, DNA sequence
ggcgcgccaggttctcctgctggctcccccacctcaacagaagaggggacaagcgaaagcgctacgcctgagagtggccctggctctgagccagccacctccggctctgaaacccctgcctcgagc

SEQ ID NO: 48 - protein, 144 aa, Artificial Sequence
  XTEN AE144-2A, protein sequence
TSTEPSEGSAPGSPAGSPTSTEEGTSTEPSEGSAPGTSTEPSEGSAPGTSESATPESGPGTSTEPSEGSAPGTSESATPESGPGSEPATSGSETPGTSTEPSEGSAPGTSTEPSEGSAPGTSESATPESGPGTSESATPESGPG

SEQ ID NO: 49 - DNA, 450 bp, Artificial Sequence
  XTEN AE144-2A, DNA sequence
ggcgcgccaaccagtacggagccgtccgaggggagcgcaccaggaagcccggctgggagcccgacttctaccgaagagggtacatctaccgaaccaagtgaaggttcagcaccaggcacctcaacagaaccctctgagggctcggcgcctggtacaagtgagtccgccaccccagaatccgggcctgggacaagcacagaaccttcggaagggagtgcccctggaacatccgaatcggcaaccccagaatcagggccaggatctgagcccgcgacttcgggctccgagacgcctgggacatccaccgagccctccgaaggatcagccccaggcaccagcacggagccctctgagggaagcgcacctggtaccagcgaaagcgcaactcccgaatcaggtcccggtacgagcgagtcggcgaccccggagagcgggccaggtgcctcgagc

SEQ ID NO: 50 - protein, 144 aa, Artificial Sequence
  XTEN AE144-3B, protein sequence
SPAGSPTSTEEGTSESATPESGPGSEPATSGSETPGTSESATPESGPGTSTEPSEGSAPGTSTEPSEGSAPGTSTEPSEGSAPGTSTEPSEGSAPGTSTEPSEGSAPGTSTEPSEGSAPGSPAGSPTSTEEGTSTEPSEGSAPG

SEQ ID NO: 51 - DNA, 450 bp, Artificial Sequence
  XTEN AE144-3B, DNA sequence
ggcgcgccaagtcccgctggaagcccaactagcaccgaagaggggacctcagagtccgccacccccgagtccggccctggctctgagcctgccactagcggctccgagactcctggcacatccgaaagcgctacacccgagagtggacccggcacctctaccgagcccagtgagggctccgcccctggaacaagcaccgagcccagcgaaggcagcgccccagggacctccacagagcccagtgaaggcagtgctcctggcaccagcaccgaaccaagcgagggctctgcacccgggacctccaccgagccaagcgaaggctctgcccctggcacttccaccgagcccagcgaaggcagcgcccctgggagccccgctggctctcccaccagcactgaggagggcacatctaccgaaccaagtgaaggctctgcaccaggtgcctcgagc

SEQ ID NO: 52 - protein, 144 aa, Artificial Sequence
  XTEN AE144-4A, protein sequence
TSESATPESGPGSEPATSGSETPGTSESATPESGPGSEPATSGSETPGTSESATPESGPGTSTEPSEGSAPGTSESATPESGPGSPAGSPTSTEEGSPAGSPTSTEEGSPAGSPTSTEEGTSESATPESGPGTSTEPSEGSAPG

SEQ ID NO: 53 - DNA, 450 bp, Artificial Sequence
  XTEN AE144-4A, DNA sequence
ggcgcgccaacgtccgaaagtgctacccctgagtcaggccctggtagtgagcctgccacaagcggaagcgaaactccggggacctcagagtctgccactcccgaatcggggccaggctctgaaccggccacttcagggagcgaaacaccaggaacatcggagagcgctaccccggagagcgggccaggaactagtactgagcctagcgagggaagtgcacctggtacaagcgagtccgccacacccgagtctggccctggctctccagcgggctcacccacgagcactgaagagggctctcccgctggcagcccaacgtcgacagaagaaggatcaccagcaggctcccccacatcaacagaggagggtacatcagaatctgctactcccgagagtggacccggtacctccactgagcccagcgaggggagtgcaccaggtgcctcgagc

SEQ ID NO: 54 - protein, 144 aa, Artificial Sequence
  XTEN AE144-5A, protein sequence
TSESATPESGPGSEPATSGSETPGTSESATPESGPGSEPATSGSETPGTSESATPESGPGTSTEPSEGSAPGSPAGSPTSTEEGTSESATPESGPGSEPATSGSETPGTSESATPESGPGSPAGSPTSTEEGSPAGSPTSTEEG

SEQ ID NO: 55 - DNA, 450 bp, Artificial Sequence; identical to SEQ ID NO: 18
  XTEN AE144-5A, DNA sequence

SEQ ID NO: 56 - protein, 144 aa, Artificial Sequence
  XTEN AE144-6B, protein sequence
TSTEPSEGSAPGTSESATPESGPGTSESATPESGPGTSESATPESGPGSEPATSGSETPGSEPATSGSETPGSPAGSPTSTEEGTSTEPSEGSAPGTSTEPSEGSAPGSEPATSGSETPGTSESATPESGPGTSTEPSEGSAPG

SEQ ID NO: 57 - DNA, 450 bp, Artificial Sequence
  XTEN AE144-6B, DNA sequence
ggcgcgccaacatctaccgagccttccgaaggctctgcccctgggacctcagaatctgcaacccctgaaagcggccctggaacctccgaaagtgccactcccgagagcggcccagggacaagcgagtcagcaacccctgagtctggacccggcagcgagcctgcaacctctggctcagagactcccggctcagaacccgctacctcaggctccgagacacccggctctcctgctgggagtcccacttccaccgaggaaggaacatccactgagcctagtgagggctctgcccctggaaccagcacagagccaagtgagggcagtgcaccaggatccgagccagcaaccagcgggtccgagactcccgggacctctgagtctgccaccccagagagcggacccggcacttcaaccgagccctccgaaggatcagcaccaggtgcctcgagc

SEQ ID NO: 58 - protein, 144 aa, Artificial Sequence
  XTEN AG144-1, protein sequence
PGSSPSASTGTGPGSSPSASTGTGPGTPGSGTASSSPGSSTPSGATGSPGSSPSASTGTGPGASPGTSSTGSPGTPGSGTASSSPGSSTPSGATGSPGTPGSGTASSSPGASPGTSSTGSPGASPGTSSTGSPGTPGSGTASSS

SEQ ID NO: 59 - DNA, 450 bp, Artificial Sequence
  XTEN AG144-1, DNA sequence
ggcgcgccacccgggtcgtccccgtcggcgtccaccggaacagggccagggtcatccccgtcagcgtcgactgggacgggacccgggacacccggttcggggactgcatcctcctcgcctggttcgtccaccccgtcaggagccacgggttcgccgggaagcagcccaagcgcatccactggtacagggcctggggcttcaccgggtacttcatccacggggtcaccgggaacgcccggatcggggacggcttcctcatcaccaggatcgtcaacaccctcgggcgcaacgggcagccccggaacccctggttcgggtacggcgtcgtcgagccccggtgcgagcccgggaacaagctcgacaggatcgcctggggcgtcacccggcacgtcgagcacaggcagccccggaacccctggatcgggaaccgcgtcgtcaagcgcctcgagc

SEQ ID NO: 60 - protein, 144 aa, Artificial Sequence
  XTEN AG144-A, protein sequence
GASPGTSSTGSPGSSPSASTGTGPGSSPSASTGTGPGTPGSGTASSSPGSSTPSGATGSPGSSPSASTGTGPGASPGTSSTGSPGTPGSGTASSSPGSSTPSGATGSPGTPGSGTASSSPGASPGTSSTGSPGASPGTSSTGSP

SEQ ID NO: 61 - DNA, 450 bp, Artificial Sequence
  XTEN AG144-A, DNA sequence
ggcgcgccaggtgcctcgccgggaacatcatcaactggttcacccgggtcatccccctcggcctcaaccgggacgggtcccggctcatcccccagcgccagcactggaacaggtcctggcactcctggttccggtacggcatcgtcatccccgggaagctcaacaccgtccggagcgacaggatcacctggctcgtcaccttcggcgtcaactggaacggggccaggggcctcacccggaacgtcctcgactgggtcgcctggtacgccgggatcaggaacggcctcatcctcgcctgggtcctcaacgccctcgggtgcgactggttcgccgggaactcctggctcggggacggcctcgtcgtcgcctggggcatcaccggggacgagctccacggggtcccctggagcgtcaccggggacctcctcgacaggtagcccggcctcgagc

SEQ ID NO: 62 - protein, 144 aa, Artificial Sequence
  XTEN AG144-B, protein sequence
GTPGSGTASSSPGSSTPSGATGSPGASPGTSSTGSPGTPGSGTASSSPGSSTPSGATGSPGSSPSASTGTGPGSSPSASTGTGPGSSTPSGATGSPGSSTPSGATGSPGASPGTSSTGSPGASPGTSSTGSPGASPGTSSTGSP

SEQ ID NO: 63 - DNA, 450 bp, Artificial Sequence
  XTEN AG144-B, DNA sequence
ggcgcgccaggtacaccgggcagcggcacggcttcgtcgtcacccggctcgtccacaccgtcgggagctacgggaagcccaggagcgtcaccgggaacgtcgtcaacggggtcaccgggtacgccaggtagcggcacggccagcagctcgccaggttcatcgaccccgtcgggagcgactgggtcgcccggatcaagcccgtcagcttccactggaacaggacccgggtcgtcgccgtcagcctcaacggggacaggacctggttcatcgacgccgtcaggggcgacaggctcgcccggatcgtcaacaccctcgggggcaacggggagccctggtgcgtcgcctggaacctcatccaccggaagcccgggggcctcgccgggtacgagctccacgggatcgcccggagcgtcccccggaacttcaagcacagggagccctgcctcgagc

SEQ ID NO: 64 - protein, 144 aa, Artificial Sequence
  XTEN AG144-C, protein sequence
GTPGSGTASSSPGASPGTSSTGSPGASPGTSSTGSPGASPGTSSTGSPGSSPSASTGTGPGTPGSGTASSSPGASPGTSSTGSPGASPGTSSTGSPGASPGTSSTGSPGSSTPSGATGSPGSSTPSGATGSPGASPGTSSTGSP

SEQ ID NO: 65 - DNA, 450 bp, Artificial Sequence
  XTEN AG144-C, DNA sequence
ggcgcgccaggtacacccggatcgggtacagcgtcatcgagccccggtgcgtcacctggtacgtcgagcacggggtcgccaggggcgtcccctgggacgtcctcaacaggctcgcccggtgcgtcacccggcacgtcgtccacgggttcacctggtagctccccttccgcgtccactggcaccgggcctggaactccggggagcggcacagcgagctcgtcgccgggagcatcgcctgggacatcgagcaccgggtcgccaggagcatcgcccggaacatccagcacaggaagccccggcgcgtcgcccgggacatcaagcacaggttccccgggatcgagcacgccgtccggagccactggatcaccagggagctcgacaccttccggcgcaacgggatcgcccggagccagcccgggtacgtcaagcactggctcccctgcctcgagc

SEQ ID NO: 66 - protein, 144 aa, Artificial Sequence
  XTEN AG144-F, protein sequence
GSSPSASTGTGPGSSPSASTGTGPGASPGTSSTGSPGASPGTSSTGSPGSSTPSGATGSPGSSPSASTGTGPGASPGTSSTGSPGSSPSASTGTGPGTPGSGTASSSPGSSTPSGATGSPGSSTPSGATGSPGASPGTSSTGSP

SEQ ID NO: 67 - DNA, 450 bp, Artificial Sequence
  XTEN AG144-F, DNA sequence
ggcgcgccaggctccagcccctccgcgagcacgggaaccggaccaggttcgtcaccctcagcatcaacggggacgggaccgggggcgtcaccaggaacgtcctccaccggctcgccgggtgcatcacccggaacgtcatcgaccggatcgccagggagctcgacgccatcaggcgcaacaggatcacctggctcaagccctagcgcgtcaaccggcacgggtccgggtgcctcccctggcacgtccagcaccggatcacccggatcgagcccatccgcctcaaccggaaccggacccggtacaccagggtcgggaacagcctcctcgtcaccaggctcctcaaccccctcgggagccacgggttcgcccggttcgtcaacgccttccggagcaactggtagccccggagcatcgccaggaacttcgagcacggggtcgcccgcctcgagc

SEQ ID NO: 68 - DNA, 4374 bp, Artificial Sequence
  coFVIII-1  DNA Sequence
atgcagattgagctgtctacttgctttttcctgtgcctgctgaggttttgcttttccgctacacgaaggtattatctgggggctgtggaactgtcttgggattacatgcagagtgacctgggagagctgccagtggacgcaaggtttccccctagagtccctaagtcattccccttcaacactagcgtggtctacaagaaaacactgttcgtggagtttactgatcacctgttcaacatcgcaaagcctaggccaccctggatgggactgctggggccaacaatccaggccgaggtgtacgacaccgtggtcattacacttaagaacatggcctcacaccccgtgagcctgcatgctgtgggcgtcagctactggaaggcttccgaaggagcagagtatgacgatcagacttcccagagagaaaaagaggacgataaggtgtttcctggcggatctcatacctacgtgtggcaggtcctgaaagagaatggccctatggcctccgaccctctgtgcctgacctactcttatctgagtcacgtggacctggtcaaggatctgaacagcggcctgatcggagccctgctggtgtgcagggaaggaagcctggctaaggagaaaacccagacactgcataagttcattctgctgttcgccgtgtttgacgaagggaaatcatggcacagcgagacaaagaatagtctgatgcaggacagggatgccgcttcagccagagcttggcccaaaatgcacactgtgaacggctacgtcaatcgctcactgcctgggctgatcggctgccaccgaaagagcgtgtattggcatgtcatcgggatgggcaccacacctgaagtgcactccattttcctggagggacatacctttctggtccgcaaccaccgacaggcttccctggagatctctccaattaccttcctgacagcacagactctgctgatggacctggggcagttcctgctgttttgccacatcagctcccaccagcatgatggcatggaggcttacgtgaaagtggactcttgtcccgaggaacctcagctgcggatgaagaacaatgaggaagcagaagactatgacgatgacctgaccgactccgagatggatgtggtccgattcgatgacgataacagcccctcctttatccagattagatctgtggccaagaaacaccctaagacatgggtccattacatcgcagccgaggaagaggactgggattatgcaccactggtgctggcaccagacgatcgctcctacaaatctcagtatctgaacaatgggccacagaggattggcagaaagtacaagaaagtgcggttcatggcatataccgatgagaccttcaagactcgcgaagccatccagcacgagagcggcatcctgggaccactgctgtacggagaagtgggagacaccctgctgatcattttcaagaaccaggccagccggccttacaatatctatccacatgggattacagatgtgcgccctctgtacagcaggagactgccaaagggcgtcaaacacctgaaggacttcccaatcctgcccggagaaatcttcaagtacaagtggactgtcaccgtcgaggatggccccactaagagcgaccctcggtgcctgacccgctactattctagtttcgtgaatatggaaagagatctggcaagcggactgatcggaccactgctgatttgttacaaagagagcgtggatcagagaggcaaccagatcatgtccgacaagcggaatgtgattctgttcagtgtctttgacgaaaacaggtcatggtacctgaccgagaacatccagagattcctgcctaatccagctggggtgcagctggaagatcctgagtttcaggcatctaacatcatgcatagtattaatggctacgtgttcgacagtttgcagctgagcgtgtgcctgcacgaggtcgcttactggtatatcctgagcattggggcacagacagatttcctgagcgtgttcttttccggctacacttttaagcataaaatggtctatgaggacacactgactctgttccccttcagcggcgaaaccgtgtttatgagcatggagaatcccggactgtggattctggggtgccacaacagcgatttcagaaatcgcggaatgactgccctgctgaaagtgtcaagctgtgacaagaacaccggggactactatgaagattcatacgaggacatcagcgcatatctgctgtccaaaaacaatgccattgaaccccggtcttttagtcagaatcctccagtgctgaagaggcaccagagggagatcacccgcactaccctgcagagtgatcaggaagagatcgactacgacgatacaatttctgtggaaatgaagaaagaggacttcgatatctatgacgaagatgagaaccagagtcctcgatcattccagaagaaaaccaggcattactttattgccgcagtggagcggctgtgggattatggcatgtcctctagtcctcacgtgctgcgaaatagggcccagtcaggaagcgtcccacagttcaagaaagtggtcttccaggagtttacagacgggtcctttactcagccactgtacaggggcgaactgaacgagcacctgggactgctggggccctatatcagagcagaagtggaggataacattatggtcaccttcagaaatcaggcctctcggccttacagtttttattcaagcctgatctcttacgaagaggaccagcgacagggagctgaaccacgaaaaaacttcgtgaagcctaatgagaccaaaacatacttttggaaggtgcagcaccatatggccccaacaaaagacgagttcgattgcaaggcatgggcctatttttctgacgtggatctggagaaggacgtgcacagtggcctgattggcccactgctggtgtgccatactaacaccctgaatccagcccacggccggcaggtcactgtccaggagttcgctctgttctttaccatctttgatgagacaaagagctggtacttcaccgaaaacatggagcgaaattgcagggctccatgtaacattcagatggaagaccccacattcaaggagaactaccgctttcatgctatcaatggatacatcatggatactctgcccgggctggtcatggcacaggaccagagaatccggtggtatctgctgagcatgggcagcaacgagaatatccactcaattcatttcagcgggcacgtgtttactgtcaggaagaaagaagagtacaagatggccctgtacaacctgtatcccggcgtgttcgaaaccgtcgagatgctgcctagcaaggccggaatctggagagtggaatgcctgattggagagcacctgcatgctgggatgtctaccctgtttctggtgtacagtaataagtgtcagacacccctgggaatggcatccgggcatatcagggatttccagattaccgcatctggacagtacggacagtgggcacctaagctggctagactgcactattccggatctatcaacgcttggtccacaaaagagcctttctcttggattaaggtggacctgctggccccaatgatcattcatggcatcaaaactcagggagctcggcagaagttctcctctctgtacatctcacagtttatcatcatgtacagcctggatgggaagaaatggcagacataccgcggcaatagcacaggaactctgatggtgttctttggcaacgtggacagcagcggaatcaagcacaacattttcaatccccctatcattgctagatacatccggctgcacccaacccattattctattcgaagtacactgaggatggaactgatgggatgcgatctgaacagttgttcaatgcccctggggatggagtccaaggcaatctctgacgcccagattaccgccagctcctacttcactaatatgtttgctacctggagcccttccaaagcaagactgcacctgcaaggccgcagcaacgcatggcgaccacaggtgaacaatcccaaggagtggttgcaggtcgattttcagaaaactatgaaggtgaccggggtcacaactcagggcgtgaaaagtctgctgacctcaatgtacgtcaaggagttcctgatctctagttcacaggacggacatcagtggacactgttctttcagaacgggaaggtgaaagtcttccagggcaatcaggattcctttacacctgtggtcaacagtctagaccctccactgctgaccagatacctgagaatccaccctcagtcctgggtgcaccagattgccctgagaatggaagtgctgggatgcgaggcccaggatctgtactga

SEQ ID NO: 69 - DNA, 577 bp, Artificial Sequence
  ET Promoter, DNA sequence
ctcgaggtcaattcacgcgagttaataattaccagcgcgggccaaataaataatccgcgaggggcaggtgacgtttgcccagcgcgcgctggtaattattaacctcgcgaatattgattcgaggccgcgattgccgcaatcgcgaggggcaggtgacctttgcccagcgcgcgttcgccccgccccggacggtatcgataagcttaggagcttgggctgcaggtcgagggcactgggaggatgttgagtaagatggaaaactactgatgacccttgcagagacagagtattaggacatgtttgaacaggggccgggcgatcagcaggtagctctagaggatccccgtctgtctgcacatttcgtagagcgagtgttccgatactctaatctccctaggcaaggttcatatttgtgtaggttacttattctccttttgttgactaagtcaataatcagaatcagcaggtttggagtcagcttggcagggatcagcagcctgggttggaaggagggggtataaaagccccttcaccaggagaagccgtcacacagatccacaagctcctgccaccatgg

SEQ ID NO: 70 - DNA, 4374 bp, Artificial Sequence; identical to SEQ ID NO: 1
  coFVIII-5

SEQ ID NO: 71 - DNA, 4374 bp, Artificial Sequence
  coFVIII-6
atgcagattgagctgtccacttgtttcttcctgtgcctcctgcgcttctgtttctccgccactcgccggtactaccttggagccgtggagctttcatgggactacatgcagagcgacctgggcgaactccccgtggatgccagattccccccccgcgtgccaaagtccttcccctttaacacctccgtggtgtacaagaaaaccctctttgtcgagttcactgaccacctgttcaacatcgccaagccgcgcccaccttggatgggcctcctgggaccgaccattcaagctgaagtgtacgacaccgtggtgatcaccctgaagaacatggcgtcccaccccgtgtccctgcatgcggtcggagtgtcctactggaaggcctccgaaggagctgagtacgacgaccagactagccagcgggaaaaggaggacgataaagtgttcccgggcggctcgcatacttacgtgtggcaagtcctgaaggaaaacggacctatggcatccgatcctctgtgcctgacttactcctacctttcccatgtggacctcgtgaaggacctgaacagcgggctgattggtgcacttctcgtgtgccgcgaaggttcgctcgctaaggaaaagacccagaccctccataagttcatccttttgttcgctgtgttcgatgaaggaaagtcatggcattccgaaactaagaactcgctgatgcaggaccgggatgccgcctcagcccgcgcctggcctaaaatgcatacagtcaacggatacgtgaatcggtcactgcccgggctcatcggttgtcacagaaagtccgtgtactggcacgtcatcggcatgggcactacgcctgaagtgcactccatcttcctggaagggcacaccttcctcgtgcgcaaccaccgccaggcctctctggaaatctccccgattacctttctgaccgcccagactctgctcatggacctggggcagttccttctcttctgccacatctccagccatcagcacgacggaatggaggcctacgtgaaggtggactcatgcccggaagaacctcagttgcggatgaagaacaacgaggaggccgaggactatgacgacgatttgactgactccgagatggacgtcgtgcggttcgatgacgacaacagccccagcttcatccagattcgcagcgtggccaagaagcaccccaaaacctgggtgcactacatcgcggccgaggaagaagattgggactacgccccgttggtgctggcacccgatgaccggtcgtacaagtcccagtatctgaacaatggtccgcagcggattggcagaaagtacaagaaagtgcggttcatggcgtacactgacgaaacgtttaagacccgggaggccattcaacatgagagcggcattctgggaccactgctgtacggagaggtcggcgataccctgctcatcatcttcaaaaaccaggcctcccggccttacaacatctaccctcacggaatcaccgacgtgcggccactctactcgcggcgcctgccgaagggcgtcaagcacctgaaagacttccctatcctgccgggcgaaatcttcaagtataagtggaccgtcaccgtggaggacgggcccaccaagagcgatcctaggtgtctgactcggtactactccagcttcgtgaacatggaacgggacctggcatcgggactcattggaccgctgctgatctgctacaaagagtcggtggatcaacgcggcaaccagatcatgtccgacaagcgcaacgtgatcctgttctccgtgtttgatgaaaacagatcctggtacctcactgaaaacatccagaggttcctcccaaaccccgcaggagtgcaactggaggaccctgagtttcaggcctcgaatatcatgcactcgattaacggttacgtgttcgactcgctgcagctgagcgtgtgcctccatgaagtcgcttactggtacattctgtccatcggcgcccagactgacttcctgagcgtgttcttttccggttacacctttaagcacaagatggtgtacgaagataccctgaccctgttccctttctccggcgaaacggtgttcatgtcgatggagaacccgggtctgtggattctgggatgccacaacagcgactttcggaaccgcggaatgactgccctgctgaaggtgtcctcatgcgacaagaacaccggagactactacgaggactcctacgaggatatctcagcctacctcctgtccaagaacaacgcgatcgagccgcgcagcttcagccagaacccgcctgtgctgaagaggcaccagcgagaaattacccggaccaccctccaatcggatcaggaggaaatcgactacgacgacaccatctcggtggaaatgaagaaggaagatttcgatatctacgacgaggacgaaaatcagtcccctcgctcattccaaaagaaaactagacactactttatcgccgcggtggaaagactgtgggactatggaatgtcatccagccctcacgtccttcggaaccgggcccagagcggatcggtgcctcagttcaagaaagtggtgttccaggagttcaccgacggcagcttcacccagccgctgtaccggggagaactgaacgaacacctgggcctgctcggtccctacatccgcgcggaagtggaggataacatcatggtgaccttccgtaaccaagcatccagaccttactccttctattcctccctgatctcatacgaggaggaccagcgccaaggcgccgagccccgcaagaacttcgtcaagcccaacgagactaagacctacttctggaaggtccaacaccatatggccccgaccaaggatgagtttgactgcaaggcctgggcctacttctccgacgtggaccttgagaaggatgtccattccggcctgatcgggccgctgctcgtgtgtcacaccaacaccctgaacccagcgcatggacgccaggtcaccgtccaggagtttgctctgttcttcaccatttttgacgaaactaagtcctggtacttcaccgagaatatggagcgaaactgtagagcgccctgcaatatccagatggaagatccgactttcaaggagaactatagattccacgccatcaacgggtacatcatggatactctgccggggctggtcatggcccaggatcagaggattcggtggtacttgctgtcaatgggatcgaacgaaaacattcactccattcacttctccggtcacgtgttcactgtgcgcaagaaggaggagtacaagatggcgctgtacaatctgtaccccggggtgttcgaaactgtggagatgctgccgtccaaggccggcatctggagagtggagtgcctgatcggagagcacctccacgcggggatgtccaccctcttcctggtgtactcgaataagtgccagaccccgctgggcatggcctcgggccacatcagagacttccagatcacagcaagcggacaatacggccaatgggcgccgaagctggcccgcttgcactactccggatcgatcaacgcatggtccaccaaggaaccgttctcgtggattaaggtggacctcctggcccctatgattatccacggaattaagacccagggcgccaggcagaagttctcctccctgtacatctcgcaattcatcatcatgtacagcctggacgggaagaagtggcagacttacaggggaaactccaccggcaccctgatggtctttttcggcaacgtggattcctccggcattaagcacaacatcttcaacccaccgatcatagccagatatattaggctccaccccactcactactcaatccgctcaactcttcggatggaactcatggggtgcgacctgaactcctgctccatgccgttggggatggaatcaaaggctattagcgacgcccagatcaccgcgagctcctacttcactaacatgttcgccacctggagcccctccaaggccaggctgcacttgcagggacggtcaaatgcctggcggccgcaagtgaacaatccgaaggaatggcttcaagtggatttccaaaagaccatgaaagtgaccggagtcaccacccagggagtgaagtcccttctgacctcgatgtatgtgaaggagttcctgattagcagcagccaggacgggcaccagtggaccctgttcttccaaaacggaaaggtcaaggtgttccaggggaaccaggactcgttcacacccgtggtgaactccctggaccccccactgctgacgcggtacttgaggattcatcctcagtcctgggtccatcagattgcattgcgaatggaagtcctgggctgcgaggcccaggacctgtactga

SEQ ID NO: 72 - DNA, 4824 bp, Artificial Sequence
  coFVIII-6-XTEN
atgcagattgagctgtccacttgtttcttcctgtgcctcctgcgcttctgtttctccgccactcgccggtactaccttggagccgtggagctttcatgggactacatgcagagcgacctgggcgaactccccgtggatgccagattccccccccgcgtgccaaagtccttcccctttaacacctccgtggtgtacaagaaaaccctctttgtcgagttcactgaccacctgttcaacatcgccaagccgcgcccaccttggatgggcctcctgggaccgaccattcaagctgaagtgtacgacaccgtggtgatcaccctgaagaacatggcgtcccaccccgtgtccctgcatgcggtcggagtgtcctactggaaggcctccgaaggagctgagtacgacgaccagactagccagcgggaaaaggaggacgataaagtgttcccgggcggctcgcatacttacgtgtggcaagtcctgaaggaaaacggacctatggcatccgatcctctgtgcctgacttactcctacctttcccatgtggacctcgtgaaggacctgaacagcgggctgattggtgcacttctcgtgtgccgcgaaggttcgctcgctaaggaaaagacccagaccctccataagttcatccttttgttcgctgtgttcgatgaaggaaagtcatggcattccgaaactaagaactcgctgatgcaggaccgggatgccgcctcagcccgcgcctggcctaaaatgcatacagtcaacggatacgtgaatcggtcactgcccgggctcatcggttgtcacagaaagtccgtgtactggcacgtcatcggcatgggcactacgcctgaagtgcactccatcttcctggaagggcacaccttcctcgtgcgcaaccaccgccaggcctctctggaaatctccccgattacctttctgaccgcccagactctgctcatggacctggggcagttccttctcttctgccacatctccagccatcagcacgacggaatggaggcctacgtgaaggtggactcatgcccggaagaacctcagttgcggatgaagaacaacgaggaggccgaggactatgacgacgatttgactgactccgagatggacgtcgtgcggttcgatgacgacaacagccccagcttcatccagattcgcagcgtggccaagaagcaccccaaaacctgggtgcactacatcgcggccgaggaagaagattgggactacgccccgttggtgctggcacccgatgaccggtcgtacaagtcccagtatctgaacaatggtccgcagcggattggcagaaagtacaagaaagtgcggttcatggcgtacactgacgaaacgtttaagacccgggaggccattcaacatgagagcggcattctgggaccactgctgtacggagaggtcggcgataccctgctcatcatcttcaaaaaccaggcctcccggccttacaacatctaccctcacggaatcaccgacgtgcggccactctactcgcggcgcctgccgaagggcgtcaagcacctgaaagacttccctatcctgccgggcgaaatcttcaagtataagtggaccgtcaccgtggaggacgggcccaccaagagcgatcctaggtgtctgactcggtactactccagcttcgtgaacatggaacgggacctggcatcgggactcattggaccgctgctgatctgctacaaagagtcggtggatcaacgcggcaaccagatcatgtccgacaagcgcaacgtgatcctgttctccgtgtttgatgaaaacagatcctggtacctcactgaaaacatccagaggttcctcccaaaccccgcaggagtgcaactggaggaccctgagtttcaggcctcgaatatcatgcactcgattaacggttacgtgttcgactcgctgcagctgagcgtgtgcctccatgaagtcgcttactggtacattctgtccatcggcgcccagactgacttcctgagcgtgttcttttccggttacacctttaagcacaagatggtgtacgaagataccctgaccctgttccctttctccggcgaaacggtgttcatgtcgatggagaacccgggtctgtggattctgggatgccacaacagcgactttcggaaccgcggaatgactgccctgctgaaggtgtcctcatgcgacaagaacaccggagactactacgaggactcctacgaggatatctcagcctacctcctgtccaagaacaacgcgatcgagccgcgcagcttcagccagaacggcgcgccaacatcagagagcgccacccctgaaagtggtcccgggagcgagccagccacatctgggtcggaaacgccaggcacaagtgagtctgcaactcccgagtccggacctggctccgagcctgccactagcggctccgagactccgggaacttccgagagcgctacaccagaaagcggacccggaaccagtaccgaacctagcgagggctctgctccgggcagcccagccggctctcctacatccacggaggagggcacttccgaatccgccaccccggagtcagggccaggatctgaacccgctacctcaggcagtgagacgccaggaacgagcgagtccgctacaccggagagtgggccagggagccctgctggatctcctacgtccactgaggaagggtcaccagcgggctcgcccaccagcactgaagaaggtgcctcgagcccgcctgtgctgaagaggcaccagcgagaaattacccggaccaccctccaatcggatcaggaggaaatcgactacgacgacaccatctcggtggaaatgaagaaggaagatttcgatatctacgacgaggacgaaaatcagtcccctcgctcattccaaaagaaaactagacactactttatcgccgcggtggaaagactgtgggactatggaatgtcatccagccctcacgtccttcggaaccgggcccagagcggatcggtgcctcagttcaagaaagtggtgttccaggagttcaccgacggcagcttcacccagccgctgtaccggggagaactgaacgaacacctgggcctgctcggtccctacatccgcgcggaagtggaggataacatcatggtgaccttccgtaaccaagcatccagaccttactccttctattcctccctgatctcatacgaggaggaccagcgccaaggcgccgagccccgcaagaacttcgtcaagcccaacgagactaagacctacttctggaaggtccaacaccatatggccccgaccaaggatgagtttgactgcaaggcctgggcctacttctccgacgtggaccttgagaaggatgtccattccggcctgatcgggccgctgctcgtgtgtcacaccaacaccctgaacccagcgcatggacgccaggtcaccgtccaggagtttgctctgttcttcaccatttttgacgaaactaagtcctggtacttcaccgagaatatggagcgaaactgtagagcgccctgcaatatccagatggaagatccgactttcaaggagaactatagattccacgccatcaacgggtacatcatggatactctgccggggctggtcatggcccaggatcagaggattcggtggtacttgctgtcaatgggatcgaacgaaaacattcactccattcacttctccggtcacgtgttcactgtgcgcaagaaggaggagtacaagatggcgctgtacaatctgtaccccggggtgttcgaaactgtggagatgctgccgtccaaggccggcatctggagagtggagtgcctgatcggagagcacctccacgcggggatgtccaccctcttcctggtgtactcgaataagtgccagaccccgctgggcatggcctcgggccacatcagagacttccagatcacagcaagcggacaatacggccaatgggcgccgaagctggcccgcttgcactactccggatcgatcaacgcatggtccaccaaggaaccgttctcgtggattaaggtggacctcctggcccctatgattatccacggaattaagacccagggcgccaggcagaagttctcctccctgtacatctcgcaattcatcatcatgtacagcctggacgggaagaagtggcagacttacaggggaaactccaccggcaccctgatggtctttttcggcaacgtggattcctccggcattaagcacaacatcttcaacccaccgatcatagccagatatattaggctccaccccactcactactcaatccgctcaactcttcggatggaactcatggggtgcgacctgaactcctgctccatgccgttggggatggaatcaaaggctattagcgacgcccagatcaccgcgagctcctacttcactaacatgttcgccacctggagcccctccaaggccaggctgcacttgcagggacggtcaaatgcctggcggccgcaagtgaacaatccgaaggaatggcttcaagtggatttccaaaagaccatgaaagtgaccggagtcaccacccagggagtgaagtcccttctgacctcgatgtatgtgaaggagttcctgattagcagcagccaggacgggcaccagtggaccctgttcttccaaaacggaaaggtcaaggtgttccaggggaaccaggactcgttcacacccgtggtgaactccctggaccccccactgctgacgcggtacttgaggattcatcctcagtcctgggtccatcagattgcattgcgaatggaagtcctgggctgcgaggcccaggacctgtactga

SEQ ID NO: 73 - protein, 12 aa, Artificial Sequence
  AD motif
GESPGGSSGSES

SEQ ID NO: 74 - protein, 12 aa, Artificial Sequence
  AD motif
GSEGSSGPGESS

SEQ ID NO: 75 - protein, 12 aa, Artificial Sequence
  AD motif
GSSESGSSEGGP

SEQ ID NO: 76 - protein, 12 aa, Artificial Sequence
  AD motif
GSGGEPSESGSS

SEQ ID NO: 77 - protein, 12 aa, Artificial Sequence
  AE, AM motif
GSPAGSPTSTEE

SEQ ID NO: 78 - protein, 12 aa, Artificial Sequence
  AE, AM, AQ motif
GSEPATSGSETP

SEQ ID NO: 79 - protein, 12 aa, Artificial Sequence
  AE, AM, AQ motif
GTSESATPESGP

SEQ ID NO: 80 - protein, 12 aa, Artificial Sequence
  AE, AM, AQ motif
GTSTEPSEGSAP

SEQ ID NO: 81 - protein, 12 aa, Artificial Sequence
  AF, AM motif
GSTSESPSGTAP

SEQ ID NO: 82 - protein, 12 aa, Artificial Sequence
  AF, AM motif
GTSTPESGSASP

SEQ ID NO: 83 - protein, 12 aa, Artificial Sequence
  AF, AM motif
GTSPSGESSTAP

SEQ ID NO: 84 - protein, 12 aa, Artificial Sequence
  AF, AM motif
GSTSSTAESPGP

SEQ ID NO: 85 - protein, 12 aa, Artificial Sequence
  AG, AM motif
GTPGSGTASSSP

SEQ ID NO: 86 - protein, 12 aa, Artificial Sequence
  AG, AM motif
GSSTPSGATGSP

SEQ ID NO: 87 - protein, 12 aa, Artificial Sequence
  AG, AM motif
GSSPSASTGTGP

SEQ ID NO: 88 - protein, 12 aa, Artificial Sequence
  AG, AM motif
GASPGTSSTGSP

SEQ ID NO: 89 - protein, 12 aa, Artificial Sequence
  AQ motif
GEPAGSPTSTSE

SEQ ID NO: 90 - protein, 12 aa, Artificial Sequence
  AQ motif
GTGEPSSTPASE

SEQ ID NO: 91 - protein, 12 aa, Artificial Sequence
  AQ motif
GSGPSTESAPTE

SEQ ID NO: 92 - protein, 12 aa, Artificial Sequence
  AQ motif
GSETPSGPSETA

SEQ ID NO: 93 - protein, 12 aa, Artificial Sequence
  AQ motif
GPSETSTSEPGA

SEQ ID NO: 94 - protein, 12 aa, Artificial Sequence
  AQ motif
GSPSEPTEGTSA

SEQ ID NO: 95 - protein, 12 aa, Artificial Sequence
  BC motif
GSGASEPTSTEP

SEQ ID NO: 96 - protein, 12 aa, Artificial Sequence
  BC motif
GSEPATSGTEPS

SEQ ID NO: 97 - protein, 12 aa, Artificial Sequence
  BC motif
GTSEPSTSEPGA

SEQ ID NO: 98 - protein, 12 aa, Artificial Sequence
  BC motif
GTSTEPSEPGSA

SEQ ID NO: 99 - protein, 12 aa, Artificial Sequence
  BD motif
GSTAGSETSTEA

SEQ ID NO: 100 - protein, 12 aa, Artificial Sequence
  BD motif
GSETATSGSETA

SEQ ID NO: 101 - protein, 12 aa, Artificial Sequence
  BD motif
GTSESATSESGA

SEQ ID NO: 102 - protein, 12 aa, Artificial Sequence
  BD motif
GTSTEASEGSAS

SEQ ID NO: 103 - protein, 1607 aa, Artificial Sequence
  coFVIII-6-XTEN Protein Sequence
MQIELSTCFFLCLLRFCFSATRRYYLGAVELSWDYMQSDLGELPVDARFPPRVPKSFPFNTSVVYKKTLFVEFTDHLFNIAKPRPPWMGLLGPTIQAEVYDTVVITLKNMASHPVSLHAVGVSYWKASEGAEYDDQTSQREKEDDKVFPGGSHTYVWQVLKENGPMASDPLCLTYSYLSHVDLVKDLNSGLIGALLVCREGSLAKEKTQTLHKFILLFAVFDEGKSWHSETKNSLMQDRDAASARAWPKMHTVNGYVNRSLPGLIGCHRKSVYWHVIGMGTTPEVHSIFLEGHTFLVRNHRQASLEISPITFLTAQTLLMDLGQFLLFCHISSHQHDGMEAYVKVDSCPEEPQLRMKNNEEAEDYDDDLTDSEMDVVRFDDDNSPSFIQIRSVAKKHPKTWVHYIAAEEEDWDYAPLVLAPDDRSYKSQYLNNGPQRIGRKYKKVRFMAYTDETFKTREAIQHESGILGPLLYGEVGDTLLIIFKNQASRPYNIYPHGITDVRPLYSRRLPKGVKHLKDFPILPGEIFKYKWTVTVEDGPTKSDPRCLTRYYSSFVNMERDLASGLIGPLLICYKESVDQRGNQIMSDKRNVILFSVFDENRSWYLTENIQRFLPNPAGVQLEDPEFQASNIMHSINGYVFDSLQLSVCLHEVAYWYILSIGAQTDFLSVFFSGYTFKHKMVYEDTLTLFPFSGETVFMSMENPGLWILGCHNSDFRNRGMTALLKVSSCDKNTGDYYEDSYEDISAYLLSKNNAIEPRSFSQNGAPTSESATPESGPGSEPATSGSETPGTSESATPESGPGSEPATSGSETPGTSESATPESGPGTSTEPSEGSAPGSPAGSPTSTEEGTSESATPESGPGSEPATSGSETPGTSESATPESGPGSPAGSPTSTEEGSPAGSPTSTEEGASSPPVLKRHQREITRTTLQSDQEEIDYDDTISVEMKKEDFDIYDEDENQSPRSFQKKTRHYFIAAVERLWDYGMSSSPHVLRNRAQSGSVPQFKKVVFQEFTDGSFTQPLYRGELNEHLGLLGPYIRAEVEDNIMVTFRNQASRPYSFYSSLISYEEDQRQGAEPRKNFVKPNETKTYFWKVQHHMAPTKDEFDCKAWAYFSDVDLEKDVHSGLIGPLLVCHTNTLNPAHGRQVTVQEFALFFTIFDETKSWYFTENMERNCRAPCNIQMEDPTFKENYRFHAINGYIMDTLPGLVMAQDQRIRWYLLSMGSNENIHSIHFSGHVFTVRKKEEYKMALYNLYPGVFETVEMLPSKAGIWRVECLIGEHLHAGMSTLFLVYSNKCQTPLGMASGHIRDFQITASGQYGQWAPKLARLHYSGSINAWSTKEPFSWIKVDLLAPMIIHGIKTQGARQKFSSLYISQFIIMYSLDGKKWQTYRGNSTGTLMVFFGNVDSSGIKHNIFNPPIIARYIRLHPTHYSIRSTLRMELMGCDLNSCSMPLGMESKAISDAQITASSYFTNMFATWSPSKARLHLQGRSNAWRPQVNNPKEWLQVDFQKTMKVTGVTTQGVKSLLTSMYVKEFLISSSQDGHQWTLFFQNGKVKVFQGNQDSFTPVVNSLDPPLLTRYLRIHPQSWVHQIALRMEVLGCEAQDLY